European Patent Application EP 4 606 886 A1, published August 27, 2025. Title: ANTIBODY COMBINATION SPECIFICALLY BINDING TO TRAIL OR FASL, AND BISPECIFIC ANTIBODY. Applicant: Beijing Solobio Genetechnology Co., Ltd. Application CN. The sequence listing filed with the application follows.

SEQUENCE LISTING (208 sequences)

SEQ ID NO: 1 - protein, 7 aa, synthetic construct
GFTFSNY

SEQ ID NO: 2 - protein, 7 aa, synthetic construct
GFNIKDT

SEQ ID NO: 3 - protein, 4 aa, synthetic construct
GGGS

SEQ ID NO: 4 - protein, 4 aa, synthetic construct
PANG

SEQ ID NO: 5 - protein, 4 aa, synthetic construct
TAMD

SEQ ID NO: 6 - protein, 7 aa, synthetic construct
YYGSSGA

SEQ ID NO: 7 - protein, 7 aa, synthetic construct
SQEISGF

SEQ ID NO: 8 - protein, 6 aa, synthetic construct
SSSVSY

SEQ ID NO: 9-10 - skipped (2 entries)

SEQ ID NO: 11 - protein, 6 aa, synthetic construct
YASYPR

SEQ ID NO: 12 - protein, 6 aa, synthetic construct
WSSYPY

SEQ ID NO: 13 - protein, 115 aa, synthetic construct
EVMLVESGGGLVQPGGSLKLSCAASGFTFSNYGMSWVRQTPEKRLEWVATISGGGSYTYYPDNLKGRFTISRENAKNTLYLQMSSLRSEDTAMYYCAAPTAMDYWGQGTSVTVSS

SEQ ID NO: 14 - protein, 115 aa, synthetic construct
EVQLVESGGGLVQPGGSLRLSCAASGFTFSNYGMSWVRQAPGKRLEWVATISGGGSYTYYPDNLKGRFTISRDNAKNSLYLQMNSLRAEDTAVYYCAAPTAMDYWGQGTLVTVSS

SEQ ID NO: 15 - protein, 118 aa, synthetic construct
EVQLQQSGAELVKPGASVKLSCTASGFNIKDTYMHWVKQRPEQGLEWIGRIRPANGNTKYDPKFQGKATVTADISSNTAYLQLSSLTSEDTAVYYCASYYYGSSGAYWGQGTLVTVSA

SEQ ID NO: 16 - protein, 118 aa, synthetic construct
EVQLVQSGAEVKKPGATVKISCKASGFNIKDTYMHWVQQAPGKGLEWIGRIRPANGNTKYDPKFQGRATVTADISTDTAYMELSSLRSEDTAVYYCASYYYGSSGAYWGQGTLVTVSS

SEQ ID NO: 17 - protein, 118 aa, synthetic construct
EVQLVQSGAEVKKPGATVKISCKASGFNIKDTYMHWVQQAPGKGLEWMGRIRPANGNTKYDPKFQGRATVTADISTDTAYMELSSLRSEDTAVYYCASYYYGSSGAYWGQGTLVTVSS

SEQ ID NO: 18 - protein, 118 aa, synthetic construct
EVQLVQSGAEVKKPGATVKISCKASGFNIKDTYMHWVQQAPGKGLEWIGRIRPANGNTKYDPKFQGRATVTADTSTDTAYMELSSLRSEDTAVYYCASYYYGSSGAYWGQGTLVTVSS

SEQ ID NO: 19 - protein, 118 aa, synthetic construct
EVQLVQSGAEVKKPGATVKISCKASGFNIKDTYMHWVQQAPGKGLEWIGRIRPANGNTKYDPKFQGRVTVTADTSTDTAYMELSSLRSEDTAVYYCASYYYGSSGAYWGQGTLVTVSS

SEQ ID NO: 20 - protein, 118 aa, synthetic construct
EVQLVQSGAEVKKPGATVKISCKASGFNIKDTYMHWVQQAPGKGLEWIGRIRPANGNTKYDPKFQGRVTITADTSTDTAYMELSSLRSEDTAVYYCASYYYGSSGAYWGQGTLVTVSS

SEQ ID NO: 21 - protein, 118 aa, synthetic construct
DVQLQESGAELVKPGASVKLSCTASGFNIKDTYMHWVKQRPEQGLEWIGRIRPANGNTKYDPKFQGRATITADTSSNTAYLQLSSLTSEDTAVYYCASYYYGSSGAYWGQGTTVTVSS

SEQ ID NO: 22 - protein, 107 aa, synthetic construct
DILLTQSPSSLSASLGERVSLTCRASQEISGFLSWLQQKPDGTIKRLIYAASTLDSGVPKRFSGSRSGSDYSLTISSLESDDFADYYCLQYASYPRTFGGGTKLEIK

SEQ ID NO: 23 - protein, 107 aa, synthetic construct
DIQLTQSPSFLSASVGDRVTITCRASQEISGFLSWLQQKPGKTIKRLIYAASTLDSGVPSRFSGSRSGSEYTLTISSLQPEDFATYYCLQYASYPRTFGGGTKVEIK

SEQ ID NO: 24 - protein, 107 aa, synthetic construct
DIQLTQSPSFLSASVGDRVTITCRASQEISGFLSWLQQKPGKTIKRLIYAASTLDSGVPSRFSGSRSGTEYTLTISSLQPEDFATYYCLQYASYPRTFGGGTKVEIK

SEQ ID NO: 25 - protein, 107 aa, synthetic construct
DIQLTQSPSFLSASVGDRVTITCRASQEISGFLSWLQQKPGKTPKRLIYAASTLDSGVPSRFSGSRSGTEYTLTISSLQPEDFATYYCLQYASYPRTFGGGTKVEIK

SEQ ID NO: 26 - protein, 107 aa, synthetic construct
DIQLTQSPSFLSASVGDRVTITCRASQEISGFLSWLQQKPGKTIKRLIYAASTLDSGVPSRFSGSRSGTEFTLTISSLQPEDFATYYCLQYASYPRTFGGGTKVEIK

SEQ ID NO: 27 - protein, 107 aa, synthetic construct
DIQLTQSPSFLSASVGDRVTITCRASQEISGFLSWLQQKPGKTPKRLIYAASTLDSGVPSRFSGSRSGTEFTLTISSLQPEDFATYYCLQYASYPRTFGGGTKVEIK

SEQ ID NO: 28 - protein, 106 aa, synthetic construct
DIVMTQSPAIMSASLGEKVTMTCSVSSSVSYMYWYQQKPGSSPRLLIYDTSSLASGVPVRFSGSGSGTSYSLTISRMEAEDAATYYCQQWSSYPYTFGGGTKLEIK

SEQ ID NO: 29 - protein, 106 aa, synthetic construct
EIVMTQSPATLSVSPGERATLSCSVSSSVSYMYWYQQKPGQSPRLLIYDTSSLASGIPARFSGSGSGTEYTLTISSLQSEDFAVYYCQQWSSYPYTFGGGTKVEIK

SEQ ID NO: 30 - protein, 106 aa, synthetic construct
EIVMTQSPATLSVSPGERATLSCSVSSSVSYMYWYQQKPGQSPRLLIYDTSSLASGIPARFSGSGSGTEFTLTISSLQSEDFAVYYCQQWSSYPYTFGGGTKVEIK

SEQ ID NO: 31 - protein, 106 aa, synthetic construct
EIVMTQSPATLSVSPGERATLSCSVSSSVSYMYWYQQKPGQAPRLLIYDTSSLASGIPARFSGSGSGTEFTLTISSLQSEDFAVYYCQQWSSYPYTFGGGTKVEIK

SEQ ID NO: 32 - protein, 106 aa, synthetic construct
QIVLTQSPAIMSASPGEKVTMTCSASSSVSYMYWYQQKPGSSPRLLIYDTSNLASGVPVRFSGSGSGTSYSLTISRMEAEDAATYYCQQWSSYPYTFGGGTKLEIK

SEQ ID NO: 33 - protein, 115 aa, synthetic construct
EVMLVESGGGLVQPGGSLKLSCAASGFTFSNYGMSWVRQTPEKCLEWVATISGGGSYTYYPDNLKGRFTISRENAKNTLYLQMSSLRSEDTAMYYCAAPTAMDYWGQGTSVTVSS

SEQ ID NO: 34 - protein, 115 aa, synthetic construct
EVQLVESGGGLVQPGGSLRLSCAASGFTFSNYGMSWVRQAPGKCLEWVATISGGGSYTYYPDNLKGRFTISRDNAKNSLYLQMNSLRAEDTAVYYCAAPTAMDYWGQGTLVTVSS

SEQ ID NO: 35 - protein, 118 aa, synthetic construct
EVQLQQSGAELVKPGASVKLSCTASGFNIKDTYMHWVKQRPEQCLEWIGRIRPANGNTKYDPKFQGKATVTADISSNTAYLQLSSLTSEDTAVYYCASYYYGSSGAYWGQGTLVTVSA

SEQ ID NO: 36 - protein, 118 aa, synthetic construct
EVQLVQSGAEVKKPGATVKISCKASGFNIKDTYMHWVQQAPGKCLEWIGRIRPANGNTKYDPKFQGRATVTADISTDTAYMELSSLRSEDTAVYYCASYYYGSSGAYWGQGTLVTVSS

SEQ ID NO: 37 - protein, 118 aa, synthetic construct
EVQLVQSGAEVKKPGATVKISCKASGFNIKDTYMHWVQQAPGKCLEWMGRIRPANGNTKYDPKFQGRATVTADISTDTAYMELSSLRSEDTAVYYCASYYYGSSGAYWGQGTLVTVSS

SEQ ID NO: 38 - protein, 118 aa, synthetic construct
EVQLVQSGAEVKKPGATVKISCKASGFNIKDTYMHWVQQAPGKCLEWIGRIRPANGNTKYDPKFQGRATVTADTSTDTAYMELSSLRSEDTAVYYCASYYYGSSGAYWGQGTLVTVSS

SEQ ID NO: 39 - protein, 118 aa, synthetic construct
EVQLVQSGAEVKKPGATVKISCKASGFNIKDTYMHWVQQAPGKCLEWIGRIRPANGNTKYDPKFQGRVTVTADTSTDTAYMELSSLRSEDTAVYYCASYYYGSSGAYWGQGTLVTVSS

SEQ ID NO: 40 - protein, 118 aa, synthetic construct
EVQLVQSGAEVKKPGATVKISCKASGFNIKDTYMHWVQQAPGKCLEWIGRIRPANGNTKYDPKFQGRVTITADTSTDTAYMELSSLRSEDTAVYYCASYYYGSSGAYWGQGTLVTVSS

SEQ ID NO: 41 - protein, 107 aa, synthetic construct
DILLTQSPSSLSASLGERVSLTCRASQEISGFLSWLQQKPDGTIKRLIYAASTLDSGVPKRFSGSRSGSDYSLTISSLESDDFADYYCLQYASYPRTFGCGTKLEIK

SEQ ID NO: 42 - protein, 107 aa, synthetic construct
DIQLTQSPSFLSASVGDRVTITCRASQEISGFLSWLQQKPGKTIKRLIYAASTLDSGVPSRFSGSRSGSEYTLTISSLQPEDFATYYCLQYASYPRTFGCGTKVEIK

SEQ ID NO: 43 - protein, 107 aa, synthetic construct
DIQLTQSPSFLSASVGDRVTITCRASQEISGFLSWLQQKPGKTIKRLIYAASTLDSGVPSRFSGSRSGTEYTLTISSLQPEDFATYYCLQYASYPRTFGCGTKVEIK

SEQ ID NO: 44 - protein, 107 aa, synthetic construct
DIQLTQSPSFLSASVGDRVTITCRASQEISGFLSWLQQKPGKTPKRLIYAASTLDSGVPSRFSGSRSGTEYTLTISSLQPEDFATYYCLQYASYPRTFGCGTKVEIK

SEQ ID NO: 45 - protein, 107 aa, synthetic construct
DIQLTQSPSFLSASVGDRVTITCRASQEISGFLSWLQQKPGKTIKRLIYAASTLDSGVPSRFSGSRSGTEFTLTISSLQPEDFATYYCLQYASYPRTFGCGTKVEIK

SEQ ID NO: 46 - protein, 107 aa, synthetic construct
DIQLTQSPSFLSASVGDRVTITCRASQEISGFLSWLQQKPGKTPKRLIYAASTLDSGVPSRFSGSRSGTEFTLTISSLQPEDFATYYCLQYASYPRTFGCGTKVEIK

SEQ ID NO: 47 - protein, 106 aa, synthetic construct
DIVMTQSPAIMSASLGEKVTMTCSVSSSVSYMYWYQQKPGSSPRLLIYDTSSLASGVPVRFSGSGSGTSYSLTISRMEAEDAATYYCQQWSSYPYTFGCGTKLEIK

SEQ ID NO: 48 - protein, 106 aa, synthetic construct
EIVMTQSPATLSVSPGERATLSCSVSSSVSYMYWYQQKPGQSPRLLIYDTSSLASGIPARFSGSGSGTEYTLTISSLQSEDFAVYYCQQWSSYPYTFGCGTKVEIK

SEQ ID NO: 49 - protein, 106 aa, synthetic construct
EIVMTQSPATLSVSPGERATLSCSVSSSVSYMYWYQQKPGQSPRLLIYDTSSLASGIPARFSGSGSGTEFTLTISSLQSEDFAVYYCQQWSSYPYTFGCGTKVEIK

SEQ ID NO: 50 - protein, 106 aa, synthetic construct
EIVMTQSPATLSVSPGERATLSCSVSSSVSYMYWYQQKPGQAPRLLIYDTSSLASGIPARFSGSGSGTEFTLTISSLQSEDFAVYYCQQWSSYPYTFGCGTKVEIK

SEQ ID NO: 51 - protein, 7 aa, synthetic construct
GFTFSSY

SEQ ID NO: 52 - protein, 7 aa, synthetic construct
GYTFTDY

SEQ ID NO: 53 - protein, 4 aa, synthetic construct
SGGG

SEQ ID NO: 54 - protein, 4 aa, synthetic construct
TYQG

SEQ ID NO: 55 - protein, 9 aa, synthetic construct
YDNYLYAMD

SEQ ID NO: 56 - protein, 8 aa, synthetic construct
PDWDYAMD

SEQ ID NO: 57 - protein, 7 aa, synthetic construct
SQTIGTW

SEQ ID NO: 58 - protein, 11 aa, synthetic construct
SQSVDYDGDSY

SEQ ID NO: 59-60 - skipped (2 entries)

SEQ ID NO: 61 - protein, 6 aa, synthetic construct
LYSTPF

SEQ ID NO: 62 - protein, 6 aa, synthetic construct
SRELPY

SEQ ID NO: 63 - protein, 120 aa, synthetic construct
DVQLQESGGGLVQPGGSRKLSCAASGFTFSSYDMSWVRQTPEKRLEWVAFISSGGGSTYYPDTVKGRFTISRDNAKNTLYLQMSSLKSEDSAMYYCGRHYDNYLYAMDYWGQGTSVTVSS

SEQ ID NO: 64 - protein, 120 aa, synthetic construct
EVQLVESGGGLVQPGGSLRLSCAASGFTFSSYDMSWVRQAPGKRLEWVAFISSGGGSTYYPDTVKGRFTISRDNAKNSLYLQMNSLRAEDTAVYYCGRHYDNYLYAMDYWGQGTLVTVSS

SEQ ID NO: 65 - protein, 120 aa, synthetic construct
EVQLVESGGGLVQPGGSLRLSCAASGFTFSSYDMSWVRQAPGKGLEWVAFISSGGGSTYYPDTVKGRFTISRDNAKNSLYLQMNSLRAEDTAVYYCGRHYDNYLYAMDYWGQGTLVTVSS

SEQ ID NO: 66 - protein, 119 aa, synthetic construct
EVQLQQSGAELVRPGVSVKISCKGSGYTFTDYTIHWVKQSHAKSLEWIGVISTYQGDASYNQKFKGKATMTVDKSSSTAYMELARLTSEDSAIYYCARFPDWDYAMDYWGQGTSVTVSS

SEQ ID NO: 67 - protein, 119 aa, synthetic construct
QVQLVQSGAEVKKPGASVKVSCKGSGYTFTDYTIHWVRQAPGQGLEWIGVISTYQGDASYNQKFKGRATMTVDKSTSTAYMELSSLRSEDTAVYYCARFPDWDYAMDYWGQGTLVTVSS

SEQ ID NO: 68 - protein, 119 aa, synthetic construct
QVQLVQSGAEVKKPGASVKVSCKASGYTFTDYTIHWVRQAPGQGLEWIGVISTYQGDASYNQKFKGRATMTVDKSTSTAYMELSSLRSEDTAVYYCARFPDWDYAMDYWGQGTLVTVSS

SEQ ID NO: 69 - protein, 119 aa, synthetic construct
QVQLVQSGAEVKKPGASVKVSCKGSGYTFTDYTIHWVRQAPGQGLEWMGVISTYQGDASYNQKFKGRATMTVDKSTSTAYMELSSLRSEDTAVYYCARFPDWDYAMDYWGQGTLVTVSS

SEQ ID NO: 70 - protein, 119 aa, synthetic construct
QVQLVQSGAEVKKPGASVKVSCKGSGYTFTDYTIHWVRQAPGQGLEWMGVISTYQGDASYNQKFKGRVTMTVDKSTSTAYMELSSLRSEDTAVYYCARFPDWDYAMDYWGQGTLVTVSS

SEQ ID NO: 71 - protein, 119 aa, synthetic construct
QVQLVQSGAEVKKPGASVKVSCKGSGYTFTDYTIHWVRQAPGQGLEWMGVISTYQGDASYNQKFKGRVTMTVDKSTSTVYMELSSLRSEDTAVYYCARFPDWDYAMDYWGQGTLVTVSS

SEQ ID NO: 72 - protein, 119 aa, synthetic construct
QVQLVQSGAEVKKPGASVKVSCKASGYTFTDYTIHWVRQAPGQGLEWMGVISTYQGDASYNQKFKGRVTMTVDTSTSTVYMELSSLRSEDTAVYYCARFPDWDYAMDYWGQGTLVTVSS

SEQ ID NO: 73 - protein, 107 aa, synthetic construct
DIVMTQSPASQSASLGESVTITCLASQTIGTWLAWYQQKPGKSPQLLIYAATSLADGVPSRFSGSGSGTKFSFKISSLQAEDFVSYYCQQLYSTPFTFGGGTKLEIK

SEQ ID NO: 74 - protein, 107 aa, synthetic construct
DIQMTQSPSSLSASVGDRVTITCLASQTIGTWLAWYQQKPGKSPKLLIYAATSLADGVPSRFSGSGSGTDFTLTISSLQPEDFATYYCQQLYSTPFTFGQGTKVEIK

SEQ ID NO: 75 - protein, 107 aa, synthetic construct
DIQMTQSPSSLSASVGDRVTITCLASQTIGTWLAWYQQKPGKAPKLLIYAATSLADGVPSRFSGSGSGTDFTLTISSLQPEDFATYYCQQLYSTPFTFGQGTKVEIK

SEQ ID NO: 76 - protein, 111 aa, synthetic construct
EIVLTQSPASLAVSLGQRATISCKASQSVDYDGDSYMNWYQQKPGQPPKLLIYAASNLESGVPARFSGSGSGTDFTLNIHPVEEEDAATYYCQHSRELPYTFGGGTKLEIK

SEQ ID NO: 77 - protein, 111 aa, synthetic construct
EIVMTQSPATLSVSPGERATLSCKASQSVDYDGDSYMNWYQQKPGQPPRLLIYAASNLESGIPARFSGSGSGTEFTLTISSLQSEDFAVYYCQHSRELPYTFGQGTKLEIK

SEQ ID NO: 78 - protein, 111 aa, synthetic construct
EIVMTQSPATLSVSPGERATLSCKASQSVDYDGDSYMNWYQQKPGQAPRLLIYAASNLESGIPARFSGSGSGTEFTLTISSLQSEDFAVYYCQHSRELPYTFGQGTKLEIK

SEQ ID NO: 79 - protein, 111 aa, synthetic construct
EIVMTQSPATLSVSPGERATLSCKASQSVDYDGDSYMNWYQQKPGQPPRLLIYAASNLESGIPARFSGSGSGTEFTLTISSLQSEDFAVYYCQQSRELPYTFGQGTKLEIK

SEQ ID NO: 80 - protein, 120 aa, synthetic construct
DVQLQESGGGLVQPGGSRKLSCAASGFTFSSYDMSWVRQTPEKCLEWVAFISSGGGSTYYPDTVKGRFTISRDNAKNTLYLQMSSLKSEDSAMYYCGRHYDNYLYAMDYWGQGTSVTVSS

SEQ ID NO: 81 - protein, 120 aa, synthetic construct
EVQLVESGGGLVQPGGSLRLSCAASGFTFSSYDMSWVRQAPGKCLEWVAFISSGGGSTYYPDTVKGRFTISRDNAKNSLYLQMNSLRAEDTAVYYCGRHYDNYLYAMDYWGQGTLVTVSS

SEQ ID NO: 82 - protein, 119 aa, synthetic construct
EVQLQQSGAELVRPGVSVKISCKGSGYTFTDYTIHWVKQSHAKCLEWIGVISTYQGDASYNQKFKGKATMTVDKSSSTAYMELARLTSEDSAIYYCARFPDWDYAMDYWGQGTSVTVSS

SEQ ID NO: 83 - protein, 119 aa, synthetic construct
QVQLVQSGAEVKKPGASVKVSCKGSGYTFTDYTIHWVRQAPGQCLEWIGVISTYQGDASYNQKFKGRATMTVDKSTSTAYMELSSLRSEDTAVYYCARFPDWDYAMDYWGQGTLVTVSS

SEQ ID NO: 84 - protein, 119 aa, synthetic construct
QVQLVQSGAEVKKPGASVKVSCKASGYTFTDYTIHWVRQAPGQCLEWIGVISTYQGDASYNQKFKGRATMTVDKSTSTAYMELSSLRSEDTAVYYCARFPDWDYAMDYWGQGTLVTVSS

SEQ ID NO: 85 - protein, 119 aa, synthetic construct
QVQLVQSGAEVKKPGASVKVSCKGSGYTFTDYTIHWVRQAPGQCLEWMGVISTYQGDASYNQKFKGRATMTVDKSTSTAYMELSSLRSEDTAVYYCARFPDWDYAMDYWGQGTLVTVSS

SEQ ID NO: 86 - protein, 119 aa, synthetic construct
QVQLVQSGAEVKKPGASVKVSCKGSGYTFTDYTIHWVRQAPGQCLEWMGVISTYQGDASYNQKFKGRVTMTVDKSTSTAYMELSSLRSEDTAVYYCARFPDWDYAMDYWGQGTLVTVSS

SEQ ID NO: 87 - protein, 119 aa, synthetic construct
QVQLVQSGAEVKKPGASVKVSCKGSGYTFTDYTIHWVRQAPGQCLEWMGVISTYQGDASYNQKFKGRVTMTVDKSTSTVYMELSSLRSEDTAVYYCARFPDWDYAMDYWGQGTLVTVSS

SEQ ID NO: 88 - protein, 119 aa, synthetic construct
QVQLVQSGAEVKKPGASVKVSCKASGYTFTDYTIHWVRQAPGQCLEWMGVISTYQGDASYNQKFKGRVTMTVDTSTSTVYMELSSLRSEDTAVYYCARFPDWDYAMDYWGQGTLVTVSS

SEQ ID NO: 89 - protein, 107 aa, synthetic construct
DIVMTQSPASQSASLGESVTITCLASQTIGTWLAWYQQKPGKSPQLLIYAATSLADGVPSRFSGSGSGTKFSFKISSLQAEDFVSYYCQQLYSTPFTFGCGTKLEIK

SEQ ID NO: 90 - protein, 107 aa, synthetic construct
DIQMTQSPSSLSASVGDRVTITCLASQTIGTWLAWYQQKPGKSPKLLIYAATSLADGVPSRFSGSGSGTDFTLTISSLQPEDFATYYCQQLYSTPFTFGCGTKVEIK

SEQ ID NO: 91 - protein, 107 aa, synthetic construct
DIQMTQSPSSLSASVGDRVTITCLASQTIGTWLAWYQQKPGKAPKLLIYAATSLADGVPSRFSGSGSGTDFTLTISSLQPEDFATYYCQQLYSTPFTFGCGTKVEIK

SEQ ID NO: 92 - protein, 111 aa, synthetic construct
EIVLTQSPASLAVSLGQRATISCKASQSVDYDGDSYMNWYQQKPGQPPKLLIYAASNLESGVPARFSGSGSGTDFTLNIHPVEEEDAATYYCQHSRELPYTFGCGTKLEIK

SEQ ID NO: 93 - protein, 111 aa, synthetic construct
EIVMTQSPATLSVSPGERATLSCKASQSVDYDGDSYMNWYQQKPGQPPRLLIYAASNLESGIPARFSGSGSGTEFTLTISSLQSEDFAVYYCQHSRELPYTFGCGTKLEIK

SEQ ID NO: 94 - protein, 111 aa, synthetic construct
EIVMTQSPATLSVSPGERATLSCKASQSVDYDGDSYMNWYQQKPGQAPRLLIYAASNLESGIPARFSGSGSGTEFTLTISSLQSEDFAVYYCQHSRELPYTFGCGTKLEIK

SEQ ID NO: 95 - protein, 111 aa, synthetic construct
EIVMTQSPATLSVSPGERATLSCKASQSVDYDGDSYMNWYQQKPGQPPRLLIYAASNLESGIPARFSGSGSGTEFTLTISSLQSEDFAVYYCQQSRELPYTFGCGTKLEIK

SEQ ID NO: 96 - protein, 330 aa, synthetic construct
ASTKGPSVFPLAPSSKSTSGGTAALGCLVKDYFPEPVTVSWNSGALTSGVHTFPAVLQSSGLYSLSSVVTVPSSSLGTQTYICNVNHKPSNTKVDKKVEPKSCDKTHTCPPCPAPELLGGPSVFLFPPKPKDTLMISRTPEVTCVVVDVSHEDPEVKFNWYVDGVEVHNAKTKPREEQYNSTYRVVSVLTVLHQDWLNGKEYKCKVSNKALPAPIEKTISKAKGQPREPQVYTLPPSREEMTKNQVSLTCLVKGFYPSDIAVEWESNGQPENNYKTTPPVLDSDGSFFLYSKLTVDKSRWQQGNVFSCSVMHEALHNHYTQKSLSLSPGK

SEQ ID NO: 97 - protein, 327 aa, synthetic construct
ASTKGPSVFPLAPCSRSTSESTAALGCLVKDYFPEPVTVSWNSGALTSGVHTFPAVLQSSGLYSLSSVVTVPSSSLGTKTYTCNVDHKPSNTKVDKRVESKYGPPCPSCPAPEFLGGPSVFLFPPKPKDTLMISRTPEVTCVVVDVSQEDPEVQFNWYVDGVEVHNAKTKPREEQFNSTYRVVSVLTVLHQDWLNGKEYKCKVSNKGLPSSIEKTISKAKGQPREPQVYTLPPSQEEMTKNQVSLTCLVKGFYPSDIAVEWESNGQPENNYKTTPPVLDSDGSFFLYSRLTVDKSRWQEGNVFSCSVMHEALHNHYTQKSLSLSLGK

SEQ ID NO: 98 - protein, 107 aa, synthetic construct [sequence omitted]

SEQ ID NO: 99 - protein, 106 aa, synthetic construct
GQPKAAPSVTLFPPSSEELQANKATLVCLISDFYPGAVTVAWKADSSPVKAGVETTTPSKQSNNKYAASSYLSLTPEQWKSHRSYSCQVTHEGSTVEKTVAPTECS

SEQ ID NO: 100 - protein, 217 aa, synthetic construct
APELLGGPSVFLFPPKPKDTLMISRTPEVTCVVVDVSHEDPEVKFNWYVDGVEVHNAKTKPREEQYNSTYRVVSVLTVLHQDWLNGKEYKCKVSNKALPAPIEKTISKAKGQPREPQVYTLPPSREEMTKNQVSLTCLVKGFYPSDIAVEWESNGQPENNYKTTPPVLDSDGSFFLYSKLTVDKSRWQQGNVFSCSVMHEALHNHYTQKSLSLSPGK

SEQ ID NO: 101 - protein, 217 aa, synthetic construct
APEFLGGPSVFLFPPKPKDTLMISRTPEVTCVVVDVSQEDPEVQFNWYVDGVEVHNAKTKPREEQFNSTYRVVSVLTVLHQDWLNGKEYKCKVSNKGLPSSIEKTISKAKGQPREPQVYTLPPSQEEMTKNQVSLTCLVKGFYPSDIAVEWESNGQPENNYKTTPPVLDSDGSFFLYSRLTVDKSRWQEGNVFSCSVMHEALHNHYTQKSLSLSLGK

SEQ ID NO: 102 - protein, 98 aa, synthetic construct
ASTKGPSVFPLAPSSKSTSGGTAALGCLVKDYFPEPVTVSWNSGALTSGVHTFPAVLQSSGLYSLSSVVTVPSSSLGTQTYICNVNHKPSNTKVDKKV

SEQ ID NO: 103 - protein, 98 aa, synthetic construct
ASTKGPSVFPLAPCSRSTSESTAALGCLVKDYFPEPVTVSWNSGALTSGVHTFPAVLQSSGLYSLSSVVTVPSSSLGTKTYTCNVDHKPSNTKVDKRV

SEQ ID NO: 104 - protein, 343 aa, synthetic construct
EVQLVESGGGLVQPGGSLRLSCAASGFTFSSYDMSWVRQAPGKRLEWVAFISSGGGSTYYPDTVKGRFTISRDNAKNSLYLQMNSLRAEDTAVYYCGRHYDNYLYAMDYWGQGTLVTVSSGGGGSGGGGSEVQLVESGGGLVQPGGSLRLSCAASGFTFSNYGMSWVRQAPGKRLEWVATISGGGSYTYYPDNLKGRFTISRDNAKNSLYLQMNSLRAEDTAVYYCAAPTAMDYWGQGTLVTVSSASTKGPSVFPLAPCSRSTSESTAALGCLVKDYFPEPVTVSWNSGALTSGVHTFPAVLQSSGLYSLSSVVTVPSSSLGTKTYTCNVDHKPSNTKVDKRV

SEQ ID NO: 105 - protein, 331 aa, synthetic construct
DIQMTQSPSSLSASVGDRVTITCLASQTIGTWLAWYQQKPGKSPKLLIYAATSLADGVPSRFSGSGSGTDFTLTISSLQPEDFATYYCQQLYSTPFTFGQGTKVEIKGGGGSGGGGSDIQLTQSPSFLSASVGDRVTITCRASQEISGFLSWLQQKPGKTIKRLIYAASTLDSGVPSRFSGSRSGSEYTLTISSLQPEDFATYYCLQYASYPRTFGGGTKVEIKRTVAAPSVFIFPPSDEQLKSGTASVVCLLNNFYPREAKVQWKVDNALQSGNSQESVTEQDSKDSTYSLSSTLTLSKADYEKHKVYACEVTHQGLSSPVTKSFNRGEC

SEQ ID NO: 106 - protein, 331 aa, synthetic construct
DIQMTQSPSSLSASVGDRVTITCLASQTIGTWLAWYQQKPGKSPKLLIYAATSLADGVPSRFSGSGSGTDFTLTISSLQPEDFATYYCQQLYSTPFTFGQGTKVEIKGGGGSGGGGSDIQLTQSPSFLSASVGDRVTITCRASQEISGFLSWLQQKPGKTIKRLIYAASTLDSGVPSRFSGSRSGTEYTLTISSLQPEDFATYYCLQYASYPRTFGGGTKVEIKRTVAAPSVFIFPPSDEQLKSGTASVVCLLNNFYPREAKVQWKVDNALQSGNSQESVTEQDSKDSTYSLSSTLTLSKADYEKHKVYACEVTHQGLSSPVTKSFNRGEC

SEQ ID NO: 107 - protein, 343 aa, synthetic construct
EVQLVESGGGLVQPGGSLRLSCAASGFTFSNYGMSWVRQAPGKRLEWVATISGGGSYTYYPDNLKGRFTISRDNAKNSLYLQMNSLRAEDTAVYYCAAPTAMDYWGQGTLVTVSSGGGGSGGGGSEVQLVESGGGLVQPGGSLRLSCAASGFTFSSYDMSWVRQAPGKRLEWVAFISSGGGSTYYPDTVKGRFTISRDNAKNSLYLQMNSLRAEDTAVYYCGRHYDNYLYAMDYWGQGTLVTVSSASTKGPSVFPLAPCSRSTSESTAALGCLVKDYFPEPVTVSWNSGALTSGVHTFPAVLQSSGLYSLSSVVTVPSSSLGTKTYTCNVDHKPSNTKVDKRV

SEQ ID NO: 108 - protein, 331 aa, synthetic construct
DIQLTQSPSFLSASVGDRVTITCRASQEISGFLSWLQQKPGKTIKRLIYAASTLDSGVPSRFSGSRSGSEYTLTISSLQPEDFATYYCLQYASYPRTFGGGTKVEIKGGGGSGGGGSDIQMTQSPSSLSASVGDRVTITCLASQTIGTWLAWYQQKPGKSPKLLIYAATSLADGVPSRFSGSGSGTDFTLTISSLQPEDFATYYCQQLYSTPFTFGQGTKVEIKRTVAAPSVFIFPPSDEQLKSGTASVVCLLNNFYPREAKVQWKVDNALQSGNSQESVTEQDSKDSTYSLSSTLTLSKADYEKHKVYACEVTHQGLSSPVTKSFNRGEC

SEQ ID NO: 109 - protein, 331 aa, synthetic construct
DIQLTQSPSFLSASVGDRVTITCRASQEISGFLSWLQQKPGKTIKRLIYAASTLDSGVPSRFSGSRSGTEYTLTISSLQPEDFATYYCLQYASYPRTFGGGTKVEIKGGGGSGGGGSDIQMTQSPSSLSASVGDRVTITCLASQTIGTWLAWYQQKPGKSPKLLIYAATSLADGVPSRFSGSGSGTDFTLTISSLQPEDFATYYCQQLYSTPFTFGQGTKVEIKRTVAAPSVFIFPPSDEQLKSGTASVVCLLNNFYPREAKVQWKVDNALQSGNSQESVTEQDSKDSTYSLSSTLTLSKADYEKHKVYACEVTHQGLSSPVTKSFNRGEC

SEQ ID NO: 110 - protein, 345 aa, synthetic construct
QVQLVQSGAEVKKPGASVKVSCKGSGYTFTDYTIHWVRQAPGQGLEWMGVISTYQGDASYNQKFKGRATMTVDKSTSTAYMELSSLRSEDTAVYYCARFPDWDYAMDYWGQGTLVTVSSGGGGSGGGGSEVQLVQSGAEVKKPGATVKISCKASGFNIKDTYMHWVQQAPGKGLEWIGRIRPANGNTKYDPKFQGRATVTADISTDTAYMELSSLRSEDTAVYYCASYYYGSSGAYWGQGTLVTVSSASTKGPSVFPLAPCSRSTSESTAALGCLVKDYFPEPVTVSWNSGALTSGVHTFPAVLQSSGLYSLSSVVTVPSSSLGTKTYTCNVDHKPSNTKVDKRV

SEQ ID NO: 111 - protein, 334 aa, synthetic construct
EIVMTQSPATLSVSPGERATLSCKASQSVDYDGDSYMNWYQQKPGQPPRLLIYAASNLESGIPARFSGSGSGTEFTLTISSLQSEDFAVYYCQQSRELPYTFGQGTKLEIKGGGGSGGGGSEIVMTQSPATLSVSPGERATLSCSVSSSVSYMYWYQQKPGQAPRLLIYDTSSLASGIPARFSGSGSGTEFTLTISSLQSEDFAVYYCQQWSSYPYTFGGGTKVEIKRTVAAPSVFIFPPSDEQLKSGTASVVCLLNNFYPREAKVQWKVDNALQSGNSQESVTEQDSKDSTYSLSSTLTLSKADYEKHKVYACEVTHQGLSSPVTKSFNRGEC

SEQ ID NO: 112 - protein, 476 aa, synthetic construct
EVQLQQSGAELVRPGVSVKISCKGSGYTFTDYTIHWVKQSHAKSLEWIGVISTYQGDASYNQKFKGKATMTVDKSSSTAYMELARLTSEDSAIYYCARFPDWDYAMDYWGQGTSVTVSSASTKGPSVFPLAPSSKSTSGGTAALGCLVKDYFPEPVTVSWNSGALTSGVHTFPAVLQSSGLYSLSSVVTVPSSSLGTQTYICNVNHKPSNTKVDKKVEPKSCGGGGSGGGGSEVQLQQSGAELVKPGASVKLSCTASGFNIKDTYMHWVKQRPEQCLEWIGRIRPANGNTKYDPKFQGKATVTADISSNTAYLQLSSLTSEDTAVYYCASYYYGSSGAYWGQGTLVTVSAGGGGSGGGGSGGGGSGGGGSDIVMTQSPAIMSASLGEKVTMTCSVSSSVSYMYWYQQKPGSSPRLLIYDTSSLASGVPVRFSGSGSGTSYSLTISRMEAEDAATYYCQQWSSYPYTFGCGTKLEIK

SEQ ID NO: 113 - protein, 218 aa, synthetic construct
EIVLTQSPASLAVSLGQRATISCKASQSVDYDGDSYMNWYQQKPGQPPKLLIYAASNLESGVPARFSGSGSGTDFTLNIHPVEEEDAATYYCQHSRELPYTFGGGTKLEIKRTVAAPSVFIFPPSDEQLKSGTASVVCLLNNFYPREAKVQWKVDNALQSGNSQESVTEQDSKDSTYSLSSTLTLSKADYEKHKVYACEVTHQGLSSPVTKSFNRGEC

SEQ ID NO: 114 - protein, 481 aa, synthetic construct
EVQLQQSGAELVKPGASVKLSCTASGFNIKDTYMHWVKQRPEQGLEWIGRIRPANGNTKYDPKFQGKATVTADISSNTAYLQLSSLTSEDTAVYYCASYYYGSSGAYWGQGTLVTVSAASTKGPSVFPLAPSSKSTSGGTAALGCLVKDYFPEPVTVSWNSGALTSGVHTFPAVLQSSGLYSLSSVVTVPSSSLGTQTYICNVNHKPSNTKVDKKVEPKSCGGGGSGGGGSEVQLQQSGAELVRPGVSVKISCKGSGYTFTDYTIHWVKQSHAKCLEWIGVISTYQGDASYNQKFKGKATMTVDKSSSTAYMELARLTSEDSAIYYCARFPDWDYAMDYWGQGTSVTVSSGGGGSGGGGSGGGGSGGGGSEIVLTQSPASLAVSLGQRATISCKASQSVDYDGDSYMNWYQQKPGQPPKLLIYAASNLESGVPARFSGSGSGTDFTLNIHPVEEEDAATYYCQHSRELPYTFGCGTKLEIK

SEQ ID NO: 115 - protein, 213 aa, synthetic construct
DIVMTQSPAIMSASLGEKVTMTCSVSSSVSYMYWYQQKPGSSPRLLIYDTSSLASGVPVRFSGSGSGTSYSLTISRMEAEDAATYYCQQWSSYPYTFGGGTKLEIKRTVAAPSVFIFPPSDEQLKSGTASVVCLLNNFYPREAKVQWKVDNALQSGNSQESVTEQDSKDSTYSLSSTLTLSKADYEKHKVYACEVTHQGLSSPVTKSFNRGEC

SEQ ID NO: 116 - protein, 475 aa, synthetic construct
EVQLVESGGGLVQPGGSLRLSCAASGFTFSSYDMSWVRQAPGKRLEWVAFISSGGGSTYYPDTVKGRFTISRDNAKNSLYLQMNSLRAEDTAVYYCGRHYDNYLYAMDYWGQGTLVTVSSASTKGPSVFPLAPSSKSTSGGTAALGCLVKDYFPEPVTVSWNSGALTSGVHTFPAVLQSSGLYSLSSVVTVPSSSLGTQTYICNVNHKPSNTKVDKKVEPKSCGGGGSGGGGSEVQLVESGGGLVQPGGSLRLSCAASGFTFSNYGMSWVRQAPGKCLEWVATISGGGSYTYYPDNLKGRFTISRDNAKNSLYLQMNSLRAEDTAVYYCAAPTAMDYWGQGTLVTVSSGGGGSGGGGSGGGGSGGGGSDIQLTQSPSFLSASVGDRVTITCRASQEISGFLSWLQQKPGKTIKRLIYAASTLDSGVPSRFSGSRSGSEYTLTISSLQPEDFATYYCLQYASYPRTFGCGTKVEIK

SEQ ID NO: 117 - protein, 475 aa, synthetic construct
EVQLVESGGGLVQPGGSLRLSCAASGFTFSSYDMSWVRQAPGKRLEWVAFISSGGGSTYYPDTVKGRFTISRDNAKNSLYLQMNSLRAEDTAVYYCGRHYDNYLYAMDYWGQGTLVTVSSASTKGPSVFPLAPSSKSTSGGTAALGCLVKDYFPEPVTVSWNSGALTSGVHTFPAVLQSSGLYSLSSVVTVPSSSLGTQTYICNVNHKPSNTKVDKKVEPKSCGGGGSGGGGSDIQLTQSPSFLSASVGDRVTITCRASQEISGFLSWLQQKPGKTIKRLIYAASTLDSGVPSRFSGSRSGSEYTLTISSLQPEDFATYYCLQYASYPRTFGCGTKVEIKGGGGSGGGGSGGGGSGGGGSEVQLVESGGGLVQPGGSLRLSCAASGFTFSNYGMSWVRQAPGKCLEWVATISGGGSYTYYPDNLKGRFTISRDNAKNSLYLQMNSLRAEDTAVYYCAAPTAMDYWGQGTLVTVSS

SEQ ID NO: 118 - protein, 475 aa, synthetic construct
EVQLVESGGGLVQPGGSLRLSCAASGFTFSSYDMSWVRQAPGKRLEWVAFISSGGGSTYYPDTVKGRFTISRDNAKNSLYLQMNSLRAEDTAVYYCGRHYDNYLYAMDYWGQGTLVTVSSASTKGPSVFPLAPSSKSTSGGTAALGCLVKDYFPEPVTVSWNSGALTSGVHTFPAVLQSSGLYSLSSVVTVPSSSLGTQTYICNVNHKPSNTKVDKKVEPKSCGGGGSGGGGSEVQLVESGGGLVQPGGSLRLSCAASGFTFSNYGMSWVRQAPGKRLEWVATISGGGSYTYYPDNLKGRFTISRDNAKNSLYLQMNSLRAEDTAVYYCAAPTAMDYWGQGTLVTVSSGGGGSGGGGSGGGGSGGGGSDIQLTQSPSFLSASVGDRVTITCRASQEISGFLSWLQQKPGKTIKRLIYAASTLDSGVPSRFSGSRSGTEYTLTISSLQPEDFATYYCLQYASYPRTFGGGTKVEIK

SEQ ID NO: 119 - protein, 214 aa, synthetic construct
DIQMTQSPSSLSASVGDRVTITCLASQTIGTWLAWYQQKPGKSPKLLIYAATSLADGVPSRFSGSGSGTDFTLTISSLQPEDFATYYCQQLYSTPFTFGQGTKVEIKRTVAAPSVFIFPPSDEQLKSGTASVVCLLNNFYPREAKVQWKVDNALQSGNSQESVTEQDSKDSTYSLSSTLTLSKADYEKHKVYACEVTHQGLSSPVTKSFNRGEC

SEQ ID NO: 120 - protein, 475 aa, synthetic construct
EVQLVESGGGLVQPGGSLRLSCAASGFTFSNYGMSWVRQAPGKRLEWVATISGGGSYTYYPDNLKGRFTISRDNAKNSLYLQMNSLRAEDTAVYYCAAPTAMDYWGQGTLVTVSSASTKGPSVFPLAPSSKSTSGGTAALGCLVKDYFPEPVTVSWNSGALTSGVHTFPAVLQSSGLYSLSSVVTVPSSSLGTQTYICNVNHKPSNTKVDKKVEPKSCGGGGSGGGGSEVQLVESGGGLVQPGGSLRLSCAASGFTFSSYDMSWVRQAPGKCLEWVAFISSGGGSTYYPDTVKGRFTISRDNAKNSLYLQMNSLRAEDTAVYYCGRHYDNYLYAMDYWGQGTLVTVSSGGGGSGGGGSGGGGSGGGGSDIQMTQSPSSLSASVGDRVTITCLASQTIGTWLAWYQQKPGKSPKLLIYAATSLADGVPSRFSGSGSGTDFTLTISSLQPEDFATYYCQQLYSTPFTFGCGTKVEIK

SEQ ID NO: 121 - protein, 214 aa, synthetic construct
DIQLTQSPSFLSASVGDRVTITCRASQEISGFLSWLQQKPGKTIKRLIYAASTLDSGVPSRFSGSRSGSEYTLTISSLQPEDFATYYCLQYASYPRTFGGGTKVEIKRTVAAPSVFIFPPSDEQLKSGTASVVCLLNNFYPREAKVQWKVDNALQSGNSQESVTEQDSKDSTYSLSSTLTLSKADYEKHKVYACEVTHQGLSSPVTKSFNRGEC

SEQ ID NO: 122 - protein, 214 aa, synthetic construct
DIQLTQSPSFLSASVGDRVTITCRASQEISGFLSWLQQKPGKTIKRLIYAASTLDSGVPSRFSGSRSGTEYTLTISSLQPEDFATYYCLQYASYPRTFGGGTKVEIKRTVAAPSVFIFPPSDEQLKSGTASVVCLLNNFYPREAKVQWKVDNALQSGNSQESVTEQDSKDSTYSLSSTLTLSKADYEKHKVYACEVTHQGLSSPVTKSFNRGEC

SEQ ID NO: 123 - protein, 481 aa, synthetic construct
EVQLVQSGAEVKKPGATVKISCKASGFNIKDTYMHWVQQAPGKGLEWIGRIRPANGNTKYDPKFQGRATVTADISTDTAYMELSSLRSEDTAVYYCASYYYGSSGAYWGQGTLVTVSSASTKGPSVFPLAPSSKSTSGGTAALGCLVKDYFPEPVTVSWNSGALTSGVHTFPAVLQSSGLYSLSSVVTVPSSSLGTQTYICNVNHKPSNTKVDKKVEPKSCGGGGSGGGGSEVQLQQSGAELVRPGVSVKISCKGSGYTFTDYTIHWVKQSHAKCLEWIGVISTYQGDASYNQKFKGKATMTVDKSSSTAYMELARLTSEDSAIYYCARFPDWDYAMDYWGQGTSVTVSSGGGGSGGGGSGGGGSGGGGSEIVLTQSPASLAVSLGQRATISCKASQSVDYDGDSYMNWYQQKPGQPPKLLIYAASNLESGVPARFSGSGSGTDFTLNIHPVEEEDAATYYCQHSRELPYTFGCGTKLEIK

SEQ ID NO: 124 - protein, 213 aa, synthetic construct
EIVMTQSPATLSVSPGERATLSCSVSSSVSYMYWYQQKPGQAPRLLIYDTSSLASGIPARFSGSGSGTEFTLTISSLQSEDFAVYYCQQWSSYPYTFGGGTKVEIKRTVAAPSVFIFPPSDEQLKSGTASVVCLLNNFYPREAKVQWKVDNALQSGNSQESVTEQDSKDSTYSLSSTLTLSKADYEKHKVYACEVTHQGLSSPVTKSFNRGEC

SEQ ID NO: 125 - protein, 226 aa, synthetic construct
EVQLQQSGAELVRPGVSVKISCKGSGYTFTDYTIHWVKQSHAKSLEWIGVISTYQGDASYNQKFKGKATMTVDKSSSTAYMELARLTSEDSAIYYCARFPDWDYAMDYWGQGTSVTVSSASVAAPSVFIFPPSDEQLKSGTASVVCLLNNFYPREAKVQWKVDNALQSGNSQESVTEQDSKDSTYSLSSTLTLSKADYEKHKVYACEVTHQGLSSPVTKSFNRGEC

SEQ ID NO: 126 - protein, 216 aa, synthetic construct
EIVLTQSPASLAVSLGQRATISCKASQSVDYDGDSYMNWYQQKPGQPPKLLIYAASNLESGVPARFSGSGSGTDFTLNIHPVEEEDAATYYCQHSRELPYTFGGGTKLEIKSSASTKGPSVFPLAPSSKSTSGGTAALGCLVKDYFPEPVTVSWNSGALTSGVHTFPAVLQSSGLYSLSSVVTVPSSSLGTQTYICNVNHKPSNTKVDKKVEPKSC

SEQ ID NO: 127 - protein, 216 aa, synthetic construct
EVQLQQSGAELVKPGASVKLSCTASGFNIKDTYMHWVKQRPEQGLEWIGRIRPANGNTKYDPKFQGKATVTADISSNTAYLQLSSLTSEDTAVYYCASYYYGSSGAYWGQGTLVTVSAASTKGPSVFPLAPSSKSTSGGTAALGCLVKDYFPEPVTVSWNSGALTSGVHTFPAVLQSSGLYSLSSVVTVPSSSLGTQTYICNVNHKPSNTKVDKKV

SEQ ID NO: 128 - protein, 216 aa, synthetic construct
EVQLQQSGAELVKPGASVKLSCTASGFNIKDTYMHWVKQRPEQGLEWIGRIRPANGNTKYDPKFQGKATVTADISSNTAYLQLSSLTSEDTAVYYCASYYYGSSGAYWGQGTLVTVSAASTKGPSVFPLAPCSRSTSESTAALGCLVKDYFPEPVTVSWNSGALTSGVHTFPAVLQSSGLYSLSSVVTVPSSSLGTKTYTCNVDHKPSNTKVDKRV

SEQ ID NO: 129 - protein, 213 aa, synthetic construct; identical to SEQ ID NO: 115

SEQ ID NO: 130 - protein, 216 aa, synthetic construct
EIVLTQSPASLAVSLGQRATISCKASQSVDYDGDSYMNWYQQKPGQPPKLLIYAASNLESGVPARFSGSGSGTDFTLNIHPVEEEDAATYYCQHSRELPYTFGGGTKLEIKSSASTKGPSVFPLAPCSRSTSESTAALGCLVKDYFPEPVTVSWNSGALTSGVHTFPAVLQSSGLYSLSSVVTVPSSSLGTKTYTCNVDHKPSNTKVDKRVESKYG

SEQ ID NO: 131 - protein, 572 aa, synthetic construct
EVQLVESGGGLVQPGGSLRLSCAASGFTFSSYDMSWVRQAPGKRLEWVAFISSGGGSTYYPDTVKGRFTISRDNAKNSLYLQMNSLRAEDTAVYYCGRHYDNYLYAMDYWGQGTLVTVSSGGGGSGGGGSEVQLVESGGGLVQPGGSLRLSCAASGFTFSNYGMSWVRQAPGKRLEWVATISGGGSYTYYPDNLKGRFTISRDNAKNSLYLQMNSLRAEDTAVYYCAAPTAMDYWGQGTLVTVSSASTKGPSVFPLAPCSRSTSESTAALGCLVKDYFPEPVTVSWNSGALTSGVHTFPAVLQSSGLYSLSSVVTVPSSSLGTKTYTCNVDHKPSNTKVDKRVESKYGPPCPPCPAPEFLGGPSVFLFPPKPKDTLMISRTPEVTCVVVDVSQEDPEVQFNWYVDGVEVHNAKTKPREEQFNSTYRVVSVLTVLHQDWLNGKEYKCKVSNKGLPSSIEKTISKAKGQPREPQVYTLPPSQEEMTKNQVSLTCLVKGFYPSDIAVEWESNGQPENNYKTTPPVLDSDGSFFLYSRLTVDKSRWQEGNVFSCSVMHEALHNHYTQKSLSLSLGK

SEQ ID NO: 132 - protein, 572 aa, synthetic construct
EVQLVESGGGLVQPGGSLRLSCAASGFTFSNYGMSWVRQAPGKRLEWVATISGGGSYTYYPDNLKGRFTISRDNAKNSLYLQMNSLRAEDTAVYYCAAPTAMDYWGQGTLVTVSSGGGGSGGGGSEVQLVESGGGLVQPGGSLRLSCAASGFTFSSYDMSWVRQAPGKRLEWVAFISSGGGSTYYPDTVKGRFTISRDNAKNSLYLQMNSLRAEDTAVYYCGRHYDNYLYAMDYWGQGTLVTVSSASTKGPSVFPLAPCSRSTSESTAALGCLVKDYFPEPVTVSWNSGALTSGVHTFPAVLQSSGLYSLSSVVTVPSSSLGTKTYTCNVDHKPSNTKVDKRVESKYGPPCPPCPAPEFLGGPSVFLFPPKPKDTLMISRTPEVTCVVVDVSQEDPEVQFNWYVDGVEVHNAKTKPREEQFNSTYRVVSVLTVLHQDWLNGKEYKCKVSNKGLPSSIEKTISKAKGQPREPQVYTLPPSQEEMTKNQVSLTCLVKGFYPSDIAVEWESNGQPENNYKTTPPVLDSDGSFFLYSRLTVDKSRWQEGNVFSCSVMHEALHNHYTQKSLSLSLGK

SEQ ID NO: 133 - protein, 574 aa, synthetic construct
QVQLVQSGAEVKKPGASVKVSCKGSGYTFTDYTIHWVRQAPGQGLEWMGVISTYQGDASYNQKFKGRATMTVDKSTSTAYMELSSLRSEDTAVYYCARFPDWDYAMDYWGQGTLVTVSSGGGGSGGGGSEVQLVQSGAEVKKPGATVKISCKASGFNIKDTYMHWVQQAPGKGLEWIGRIRPANGNTKYDPKFQGRATVTADISTDTAYMELSSLRSEDTAVYYCASYYYGSSGAYWGQGTLVTVSSASTKGPSVFPLAPCSRSTSESTAALGCLVKDYFPEPVTVSWNSGALTSGVHTFPAVLQSSGLYSLSSVVTVPSSSLGTKTYTCNVDHKPSNTKVDKRVESKYGPPCPPCPAPEFLGGPSVFLFPPKPKDTLMISRTPEVTCVVVDVSQEDPEVQFNWYVDGVEVHNAKTKPREEQFNSTYRVVSVLTVLHQDWLNGKEYKCKVSNKGLPSSIEKTISKAKGQPREPQVYTLPPSQEEMTKNQVSLTCLVKGFYPSDIAVEWESNGQPENNYKTTPPVLDSDGSFFLYSRLTVDKSRWQEGNVFSCSVMHEALHNHYTQKSLSLSLGK

SEQ ID NO: 134 - protein, 713 aa, synthetic construct
EVQLQQSGAELVRPGVSVKISCKGSGYTFTDYTIHWVKQSHAKSLEWIGVISTYQGDASYNQKFKGKATMTVDKSSSTAYMELARLTSEDSAIYYCARFPDWDYAMDYWGQGTSVTVSSASTKGPSVFPLAPSSKSTSGGTAALGCLVKDYFPEPVTVSWNSGALTSGVHTFPAVLQSSGLYSLSSVVTVPSSSLGTQTYICNVNHKPSNTKVDKKVEPKSCGGGGSGGGGSEVQLQQSGAELVKPGASVKLSCTASGFNIKDTYMHWVKQRPEQCLEWIGRIRPANGNTKYDPKFQGKATVTADISSNTAYLQLSSLTSEDTAVYYCASYYYGSSGAYWGQGTLVTVSAGGGGSGGGGSGGGGSGGGGSDIVMTQSPAIMSASLGEKVTMTCSVSSSVSYMYWYQQKPGSSPRLLIYDTSSLASGVPVRFSGSGSGTSYSLTISRMEAEDAATYYCQQWSSYPYTFGCGTKLEIKGGGGSGGGGSDKTHTCPPCPAPELLGGPSVFLFPPKPKDTLMISRTPEVTCVVVDVSHEDPEVKFNWYVDGVEVHNAKTKPREEQYNSTYRVVSVLTVLHQDWLNGKEYKCKVSNKALPAPIEKTISKAKGQPREPQVYTLPPSREEMTKNQVSLTCLVKGFYPSDIAVEWESNGQPENNYKTTPPVLDSDGSFFLYSKLTVDKSRWQQGNVFSCSVMHEALHNHYTQKSLSLSPGK

SEQ ID NO: 135 - protein, 715 aa, synthetic construct
EVQLQQSGAELVRPGVSVKISCKGSGYTFTDYTIHWVKQSHAKSLEWIGVISTYQGDASYNQKFKGKATMTVDKSSSTAYMELARLTSEDSAIYYCARFPDWDYAMDYWGQGTSVTVSSASTKGPSVFPLAPSSKSTSGGTAALGCLVKDYFPEPVTVSWNSGALTSGVHTFPAVLQSSGLYSLSSVVTVPSSSLGTQTYICNVNHKPSNTKVDKKVEPKSCGGGGSGGGGSEVQLQQSGAELVKPGASVKLSCTASGFNIKDTYMHWVKQRPEQCLEWIGRIRPANGNTKYDPKFQGKATVTADISSNTAYLQLSSLTSEDTAVYYCASYYYGSSGAYWGQGTLVTVSAGGGGSGGGGSGGGGSGGGGSDIVMTQSPAIMSASLGEKVTMTCSVSSSVSYMYWYQQKPGSSPRLLIYDTSSLASGVPVRFSGSGSGTSYSLTISRMEAEDAATYYCQQWSSYPYTFGCGTKLEIKGGGGSGGGGSESKYGPPCPPCPAPEFLGGPSVFLFPPKPKDTLMISRTPEVTCVVVDVSQEDPEVQFNWYVDGVEVHNAKTKPREEQFNSTYRVVSVLTVLHQDWLNGKEYKCKVSNKGLPSSIEKTISKAKGQPREPQVYTLPPSQEEMTKNQVSLTCLVKGFYPSDIAVEWESNGQPENNYKTTPPVLDSDGSFFLYSRLTVDKSRWQEGNVFSCSVMHEALHNHYTQKSLSLSLGK

SEQ ID NO: 136 - protein, 718 aa, synthetic construct
EVQLQQSGAELVKPGASVKLSCTASGFNIKDTYMHWVKQRPEQGLEWIGRIRPANGNTKYDPKFQGKATVTADISSNTAYLQLSSLTSEDTAVYYCASYYYGSSGAYWGQGTLVTVSAASTKGPSVFPLAPSSKSTSGGTAALGCLVKDYFPEPVTVSWNSGALTSGVHTFPAVLQSSGLYSLSSVVTVPSSSLGTQTYICNVNHKPSNTKVDKKVEPKSCGGGGSGGGGSEVQLQQSGAELVRPGVSVKISCKGSGYTFTDYTIHWVKQSHAKCLEWIGVISTYQGDASYNQKFKGKATMTVDKSSSTAYMELARLTSEDSAIYYCARFPDWDYAMDYWGQGTSVTVSSGGGGSGGGGSGGGGSGGGGSEIVLTQSPASLAVSLGQRATISCKASQSVDYDGDSYMNWYQQKPGQPPKLLIYAASNLESGVPARFSGSGSGTDFTLNIHPVEEEDAATYYCQHSRELPYTFGCGTKLEIKGGGGSGGGGSDKTHTCPPCPAPELLGGPSVFLFPPKPKDTLMISRTPEVTCVVVDVSHEDPEVKFNWYVDGVEVHNAKTKPREEQYNSTYRVVSVLTVLHQDWLNGKEYKCKVSNKALPAPIEKTISKAKGQPREPQVYTLPPSREEMTKNQVSLTCLVKGFYPSDIAVEWESNGQPENNYKTTPPVLDSDGSFFLYSKLTVDKSRWQQGNVFSCSVMHEALHNHYTQKSLSLSPGK

SEQ ID NO: 137 - protein, 720 aa, synthetic construct
EVQLQQSGAELVKPGASVKLSCTASGFNIKDTYMHWVKQRPEQGLEWIGRIRPANGNTKYDPKFQGKATVTADISSNTAYLQLSSLTSEDTAVYYCASYYYGSSGAYWGQGTLVTVSAASTKGPSVFPLAPSSKSTSGGTAALGCLVKDYFPEPVTVSWNSGALTSGVHTFPAVLQSSGLYSLSSVVTVPSSSLGTQTYICNVNHKPSNTKVDKKVEPKSCGGGGSGGGGSEVQLQQSGAELVRPGVSVKISCKGSGYTFTDYTIHWVKQSHAKCLEWIGVISTYQGDASYNQKFKGKATMTVDKSSSTAYMELARLTSEDSAIYYCARFPDWDYAMDYWGQGTSVTVSSGGGGSGGGGSGGGGSGGGGSEIVLTQSPASLAVSLGQRATISCKASQSVDYDGDSYMNWYQQKPGQPPKLLIYAASNLESGVPARFSGSGSGTDFTLNIHPVEEEDAATYYCQHSRELPYTFGCGTKLEIKGGGGSGGGGSESKYGPPCPPCPAPEFLGGPSVFLFPPKPKDTLMISRTPEVTCVVVDVSQEDPEVQFNWYVDGVEVHNAKTKPREEQFNSTYRVVSVLTVLHQDWLNGKEYKCKVSNKGLPSSIEKTISKAKGQPREPQVYTLPPSQEEMTKNQVSLTCLVKGFYPSDIAVEWESNGQPENNYKTTPPVLDSDGSFFLYSRLTVDKSRWQEGNVFSCSVMHEALHNHYTQKSLSLSLGK

SEQ ID NO: 138 - protein, 714 aa, synthetic construct
EVQLVESGGGLVQPGGSLRLSCAASGFTFSSYDMSWVRQAPGKRLEWVAFISSGGGSTYYPDTVKGRFTISRDNAKNSLYLQMNSLRAEDTAVYYCGRHYDNYLYAMDYWGQGTLVTVSSASTKGPSVFPLAPSSKSTSGGTAALGCLVKDYFPEPVTVSWNSGALTSGVHTFPAVLQSSGLYSLSSVVTVPSSSLGTQTYICNVNHKPSNTKVDKKVEPKSCGGGGSGGGGSEVQLVESGGGLVQPGGSLRLSCAASGFTFSNYGMSWVRQAPGKCLEWVATISGGGSYTYYPDNLKGRFTISRDNAKNSLYLQMNSLRAEDTAVYYCAAPTAMDYWGQGTLVTVSSGGGGSGGGGSGGGGSGGGGSDIQLTQSPSFLSASVGDRVTITCRASQEISGFLSWLQQKPGKTIKRLIYAASTLDSGVPSRFSGSRSGSEYTLTISSLQPEDFATYYCLQYASYPRTFGCGTKVEIKGGGGSGGGGSESKYGPPCPPCPAPEFLGGPSVFLFPPKPKDTLMISRTPEVTCVVVDVSQEDPEVQFNWYVDGVEVHNAKTKPREEQFNSTYRVVSVLTVLHQDWLNGKEYKCKVSNKGLPSSIEKTISKAKGQPREPQVYTLPPSQEEMTKNQVSLTCLVKGFYPSDIAVEWESNGQPENNYKTTPPVLDSDGSFFLYSRLTVDKSRWQEGNVFSCSVMHEALHNHYTQKSLSLSLGK

SEQ ID NO: 139 - protein, 714 aa, synthetic construct
EVQLVESGGGLVQPGGSLRLSCAASGFTFSSYDMSWVRQAPGKRLEWVAFISSGGGSTYYPDTVKGRFTISRDNAKNSLYLQMNSLRAEDTAVYYCGRHYDNYLYAMDYWGQGTLVTVSSASTKGPSVFPLAPSSKSTSGGTAALGCLVKDYFPEPVTVSWNSGALTSGVHTFPAVLQSSGLYSLSSVVTVPSSSLGTQTYICNVNHKPSNTKVDKKVEPKSCGGGGSGGGGSDIQLTQSPSFLSASVGDRVTITCRASQEISGFLSWLQQKPGKTIKRLIYAASTLDSGVPSRFSGSRSGSEYTLTISSLQPEDFATYYCLQYASYPRTFGCGTKVEIKGGGGSGGGGSGGGGSGGGGSEVQLVESGGGLVQPGGSLRLSCAASGFTFSNYGMSWVRQAPGKCLEWVATISGGGSYTYYPDNLKGRFTISRDNAKNSLYLQMNSLRAEDTAVYYCAAPTAMDYWGQGTLVTVSSGGGGSGGGGSESKYGPPCPPCPAPEFLGGPSVFLFPPKPKDTLMISRTPEVTCVVVDVSQEDPEVQFNWYVDGVEVHNAKTKPREEQFNSTYRVVSVLTVLHQDWLNGKEYKCKVSNKGLPSSIEKTISKAKGQPREPQVYTLPPSQEEMTKNQVSLTCLVKGFYPSDIAVEWESNGQPENNYKTTPPVLDSDGSFFLYSRLTVDKSRWQEGNVFSCSVMHEALHNHYTQKSLSLSLGK

SEQ ID NO: 140 - protein, 714 aa, synthetic construct
EVQLVESGGGLVQPGGSLRLSCAASGFTFSSYDMSWVRQAPGKRLEWVAFISSGGGSTYYPDTVKGRFTISRDNAKNSLYLQMNSLRAEDTAVYYCGRHYDNYLYAMDYWGQGTLVTVSSASTKGPSVFPLAPSSKSTSGGTAALGCLVKDYFPEPVTVSWNSGALTSGVHTFPAVLQSSGLYSLSSVVTVPSSSLGTQTYICNVNHKPSNTKVDKKVEPKSCGGGGSGGGGSEVQLVESGGGLVQPGGSLRLSCAASGFTFSNYGMSWVRQAPGKRLEWVATISGGGSYTYYPDNLKGRFTISRDNAKNSLYLQMNSLRAEDTAVYYCAAPTAMDYWGQGTLVTVSSGGGGSGGGGSGGGGSGGGGSDIQLTQSPSFLSASVGDRVTITCRASQEISGFLSWLQQKPGKTIKRLIYAASTLDSGVPSRFSGSRSGTEYTLTISSLQPEDFATYYCLQYASYPRTFGGGTKVEIKGGGGSGGGGSESKYGPPCPPCPAPEFLGGPSVFLFPPKPKDTLMISRTPEVTCVVVDVSQEDPEVQFNWYVDGVEVHNAKTKPREEQFNSTYRVVSVLTVLHQDWLNGKEYKCKVSNKGLPSSIEKTISKAKGQPREPQVYTLPPSQEEMTKNQVSLTCLVKGFYPSDIAVEWESNGQPENNYKTTPPVLDSDGSFFLYSRLTVDKSRWQEGNVFSCSVMHEALHNHYTQKSLSLSLGK

SEQ ID NO: 141 - protein, 714 aa, synthetic construct
EVQLVESGGGLVQPGGSLRLSCAASGFTFSNYGMSWVRQAPGKRLEWVATISGGGSYTYYPDNLKGRFTISRDNAKNSLYLQMNSLRAEDTAVYYCAAPTAMDYWGQGTLVTVSSASTKGPSVFPLAPSSKSTSGGTAALGCLVKDYFPEPVTVSWNSGALTSGVHTFPAVLQSSGLYSLSSVVTVPSSSLGTQTYICNVNHKPSNTKVDKKVEPKSCGGGGSGGGGSEVQLVESGGGLVQPGGSLRLSCAASGFTFSSYDMSWVRQAPGKCLEWVAFISSGGGSTYYPDTVKGRFTISRDNAKNSLYLQMNSLRAEDTAVYYCGRHYDNYLYAMDYWGQGTLVTVSSGGGGSGGGGSGGGGSGGGGSDIQMTQSPSSLSASVGDRVTITCLASQTIGTWLAWYQQKPGKSPKLLIYAATSLADGVPSRFSGSGSGTDFTLTISSLQPEDFATYYCQQLYSTPFTFGCGTKVEIKGGGGSGGGGSESKYGPPCPPCPAPEFLGGPSVFLFPPKPKDTLMISRTPEVTCVVVDVSQEDPEVQFNWYVDGVEVHNAKTKPREEQFNSTYRVVSVLTVLHQDWLNGKEYKCKVSNKGLPSSIEKTISKAKGQPREPQVYTLPPSQEEMTKNQVSLTCLVKGFYPSDIAVEWESNGQPENNYKTTPPVLDSDGSFFLYSRLTVDKSRWQEGNVFSCSVMHEALHNHYTQKSLSLSLGK

SEQ ID NO: 142 - protein, 720 aa, synthetic construct
EVQLVQSGAEVKKPGATVKISCKASGFNIKDTYMHWVQQAPGKGLEWIGRIRPANGNTKYDPKFQGRATVTADISTDTAYMELSSLRSEDTAVYYCASYYYGSSGAYWGQGTLVTVSSASTKGPSVFPLAPSSKSTSGGTAALGCLVKDYFPEPVTVSWNSGALTSGVHTFPAVLQSSGLYSLSSVVTVPSSSLGTQTYICNVNHKPSNTKVDKKVEPKSCGGGGSGGGGSEVQLQQSGAELVRPGVSVKISCKGSGYTFTDYTIHWVKQSHAKCLEWIGVISTYQGDASYNQKFKGKATMTVDKSSSTAYMELARLTSEDSAIYYCARFPDWDYAMDYWGQGTSVTVSSGGGGSGGGGSGGGGSGGGGSEIVLTQSPASLAVSLGQRATISCKASQSVDYDGDSYMNWYQQKPGQPPKLLIYAASNLESGVPARFSGSGSGTDFTLNIHPVEEEDAATYYCQHSRELPYTFGCGTKLEIKGGGGSGGGGSESKYGPPCPPCPAPEFLGGPSVFLFPPKPKDTLMISRTPEVTCVVVDVSQEDPEVQFNWYVDGVEVHNAKTKPREEQFNSTYRVVSVLTVLHQDWLNGKEYKCKVSNKGLPSSIEKTISKAKGQPREPQVYTLPPSQEEMTKNQVSLTCLVKGFYPSDIAVEWESNGQPENNYKTTPPVLDSDGSFFLYSRLTVDKSRWQEGNVFSCSVMHEALHNHYTQKSLSLSLGK

SEQ ID NO: 143 - protein, 453 aa, synthetic construct
EVQLQQSGAELVRPGVSVKISCKGSGYTFTDYTIHWVKQSHAKSLEWIGVISTYQGDASYNQKFKGKATMTVDKSSSTAYMELARLTSEDSAIYYCARFPDWDYAMDYWGQGTSVTVSSASVAAPSVFIFPPSDEQLKSGTASVVCLLNNFYPREAKVQWKVDNALQSGNSQESVTEQDSKDSTYSLSSTLTLSKADYEKHKVYACEVTHQGLSSPVTKSFNRGECDKTHTCPPCPAPELLGGPSVFLFPPKPKDTLMISRTPEVTCVVVDVSHEDPEVKFNWYVDGVEVHNAKTKPREEQYNSTYRVVSVLTVLHQDWLNGKEYKCKVSNKALPAPIEKTISKAKGQPREPQVCTLPPSRDELTKNQVSLSCAVKGFYPSDIAVEWESNGQPENNYKTTPPVLDSDGSFFLVSKLTVDKSRWQQGNVFSCSVMHEALHNHYTQKSLSLSPGK

SEQ ID NO: 144 - protein, 448 aa, synthetic construct
EVQLQQSGAELVKPGASVKLSCTASGFNIKDTYMHWVKQRPEQGLEWIGRIRPANGNTKYDPKFQGKATVTADISSNTAYLQLSSLTSEDTAVYYCASYYYGSSGAYWGQGTLVTVSAASTKGPSVFPLAPSSKSTSGGTAALGCLVKDYFPEPVTVSWNSGALTSGVHTFPAVLQSSGLYSLSSVVTVPSSSLGTQTYICNVNHKPSNTKVDKKVEPKSCDKTHTCPPCPAPELLGGPSVFLFPPKPKDTLMISRTPEVTCVVVDVSHEDPEVKFNWYVDGVEVHNAKTKPREEQYNSTYRVVSVLTVLHQDWLNGKEYKCKVSNKALPAPIEKTISKAKGQPREPQVYTLPPCRDELTKNQVSLWCLVKGFYPSDIAVEWESNGQPENNYKTTPPVLDSDGSFFLYSKLTVDKSRWQQGNVFSCSVMHEALHNHYTQKSLSLSPGK

SEQ ID NO: 145 - protein, 455 aa, synthetic construct
EVQLQQSGAELVRPGVSVKISCKGSGYTFTDYTIHWVKQSHAKSLEWIGVISTYQGDASYNQKFKGKATMTVDKSSSTAYMELARLTSEDSAIYYCARFPDWDYAMDYWGQGTSVTVSSASVAAPSVFIFPPSDEQLKSGTASVVCLLNNFYPREAKVQWKVDNALQSGNSQESVTEQDSKDSTYSLSSTLTLSKADYEKHKVYACEVTHQGLSSPVTKSFNRGECESKYGPPCPPCPAPEFLGGPSVFLFPPKPKDTLMISRTPEVTCVVVDVSQEDPEVQFNWYVDGVEVHNAKTKPREEQFNSTYRVVSVLTVLHQDWLNGKEYKCKVSNKGLPSSIEKTISKAKGQPREPQVCTLPPSQEEMTKNQVSLSCAVKGFYPSDIAVEWESNGQPENNYKTTPPVLDSDGSFFLVSRLTVDKSRWQEGNVFSCSVMHEALHNHYTQKSLSLSLGK

SEQ ID NO: 146 - protein, 445 aa, synthetic construct
EVQLQQSGAELVKPGASVKLSCTASGFNIKDTYMHWVKQRPEQGLEWIGRIRPANGNTKYDPKFQGKATVTADISSNTAYLQLSSLTSEDTAVYYCASYYYGSSGAYWGQGTLVTVSAASTKGPSVFPLAPCSRSTSESTAALGCLVKDYFPEPVTVSWNSGALTSGVHTFPAVLQSSGLYSLSSVVTVPSSSLGTKTYTCNVDHKPSNTKVDKRVESKYGPPCPPCPAPEFLGGPSVFLFPPKPKDTLMISRTPEVTCVVVDVSQEDPEVQFNWYVDGVEVHNAKTKPREEQFNSTYRVVSVLTVLHQDWLNGKEYKCKVSNKGLPSSIEKTISKAKGQPREPQVYTLPPCQEEMTKNQVSLWCLVKGFYPSDIAVEWESNGQPENNYKTTPPVLDSDGSFFLYSRLTVDKSRWQEGNVFSCSVMHEALHNHYTQKSLSLSLGK

SEQ ID NO: 147 - protein, 10 aa, synthetic construct
GGGGSGGGGS

SEQ ID NO: 148 - protein, 20 aa, synthetic construct
GGGGSGGGGSGGGGSGGGGS

SEQ ID NO: 149 - protein, 15 aa, synthetic construct
GGGGSGGGGSGGGGS

SEQ ID NO: 150 - protein, 6 aa, synthetic construct
ASTKGP

SEQ ID NO: 151 - protein, 5 aa, synthetic construct
TVAAP

SEQ ID NO: 152 - protein, 17 aa, synthetic construct
EPKSDKTGGGGSGGGGS

SEQ ID NO: 153 - protein, 18 aa, synthetic construct
EPKSCGKTGGGGSGGGGS

SEQ ID NO: 154 - protein, 15 aa, synthetic construct
EPKSCGGGGSGGGGS

SEQ ID NO: 155 - protein, 24 aa, synthetic construct
GGGGSGGGGSEPKSDKTHTCPPCP

SEQ ID NO: 156 - protein, 15 aa, synthetic construct
GGGGSGGGGSCPPCP

SEQ ID NO: 157 - protein, 20 aa, synthetic construct
GGGGSGGGGSDKTHTCPPCP

SEQ ID NO: 158 - protein, 20 aa, synthetic construct
GKPGSGKPGSGKPGSGKPGS

SEQ ID NO: 159 - protein, 15 aa, synthetic construct
GGGGSGGGGTGGGGS

SEQ ID NO: 160 - protein, 22 aa, synthetic construct
GGGGSGGGGSESKYGPPCPPCP

SEQ ID NO: 161 - protein, 4 aa, synthetic construct
PANA

SEQ ID NO: 162 - protein, 11 aa, synthetic construct
SQSVDYEGDSY

SEQ ID NO: 163 - protein, 120 aa, synthetic construct; identical to SEQ ID NO: 64

SEQ ID NO: 164 - protein, 115 aa, synthetic construct; identical to SEQ ID NO: 34

SEQ ID NO: 165 - protein, 119 aa, synthetic construct; identical to SEQ ID NO: 69

SEQ ID NO: 166 - protein, 118 aa, synthetic construct
EVQLVQSGAEVKKPGATVKISCKASGFNIKDTYMHWVQQAPGKGLEWIGRIRPANANAKYDPKFQGRATVTADISTDTAYMELSSLRSEDTAVYYCASYYYGSSGAYWGQGTLVTVSS

SEQ ID NO: 167 - protein, 107 aa, synthetic construct
DIQMTQSPSSLSASVGDRVTITCLASQTIGTWLAWYQQKPGKSPKLLIYAATSLASGVPSRFSGSGSGTDFTLTISSLQPEDFATYYCQQLYSTPFTFGQGTKVEIK

SEQ ID NO: 168 - protein, 107 aa, synthetic construct
DIQLTQSPSFLSASVGDRVTITCRASQEISGFLSWLQQKPGKTIKRLIYAASTLDTGVPSRFSGSRSGSEYTLTISSLQPEDFATYYCLQYASYPRTFGCGTKVEIK

SEQ ID NO: 169 - protein, 111 aa, synthetic construct
EIVMTQSPATLSVSPGERATLSCKASQSVDYEGDSYMNWYQQKPGQPPRLLIYAASNLESGIPARFSGSGSGTEFTLTISSLQSEDFAVYYCQQSRELPYTFGQGTKLEIK

SEQ ID NO: 170 - protein, 106 aa, synthetic construct; identical to SEQ ID NO: 31

SEQ ID NO: 171 - protein, 475 aa, synthetic construct
EVQLVESGGGLVQPGGSLRLSCAASGFTFSSYDMSWVRQAPGKRLEWVAFISSGGGSTYYPDTVKGRFTISRDNAKNSLYLQMNSLRAEDTAVYYCGRHYDNYLYAMDYWGQGTLVTVSSASTKGPSVFPLAPSSKSTSGGTAALGCLVKDYFPEPVTVSWNSGALTSGVHTFPAVLQSSGLYSLSSVVTVPSSSLGTQTYICNVNHKPSNTKVDKKVEPKSCGGGGSGGGGSEVQLVESGGGLVQPGGSLRLSCAASGFTFSNYGMSWVRQAPGKCLEWVATISGGGSYTYYPDNLKGRFTISRDNAKNSLYLQMNSLRAEDTAVYYCAAPTAMDYWGQGTLVTVSSGGGGSGGGGSGGGGSGGGGSDIQLTQSPSFLSASVGDRVTITCRASQEISGFLSWLQQKPGKTIKRLIYAASTLDTGVPSRFSGSRSGSEYTLTISSLQPEDFATYYCLQYASYPRTFGCGTKVEIK

SEQ ID NO: 172 - protein, 345 aa, synthetic construct
QVQLVQSGAEVKKPGASVKVSCKGSGYTFTDYTIHWVRQAPGQGLEWMGVISTYQGDASYNQKFKGRATMTVDKSTSTAYMELSSLRSEDTAVYYCARFPDWDYAMDYWGQGTLVTVSSGGGGSGGGGSEVQLVQSGAEVKKPGATVKISCKASGFNIKDTYMHWVQQAPGKGLEWIGRIRPANANAKYDPKFQGRATVTADISTDTAYMELSSLRSEDTAVYYCASYYYGSSGAYWGQGTLVTVSSASTKGPSVFPLAPCSRSTSESTAALGCLVKDYFPEPVTVSWNSGALTSGVHTFPAVLQSSGLYSLSSVVTVPSSSLGTKTYTCNVDHKPSNTKVDKRV

SEQ ID NO: 173 - protein, 214 aa, synthetic construct
DIQMTQSPSSLSASVGDRVTITCLASQTIGTWLAWYQQKPGKSPKLLIYAATSLASGVPSRFSGSGSGTDFTLTISSLQPEDFATYYCQQLYSTPFTFGQGTKVEIKRTVAAPSVFIFPPSDEQLKSGTASVVCLLNNFYPREAKVQWKVDNALQSGNSQESVTEQDSKDSTYSLSSTLTLSKADYEKHKVYACEVTHQGLSSPVTKSFNRGEC

SEQ ID NO: 174 - protein, 334 aa, synthetic construct
EIVMTQSPATLSVSPGERATLSCKASQSVDYEGDSYMNWYQQKPGQPPRLLIYAASNLESGIPARFSGSGSGTEFTLTISSLQSEDFAVYYCQQSRELPYTFGQGTKLEIKGGGGSGGGGSEIVMTQSPATLSVSPGERATLSCSVSSSVSYMYWYQQKPGQAPRLLIYDTSSLASGIPARFSGSGSGTEFTLTISSLQSEDFAVYYCQQWSSYPYTFGGGTKVEIKRTVAAPSVFIFPPSDEQLKSGTASVVCLLNNFYPREAKVQWKVDNALQSGNSQESVTEQDSKDSTYSLSSTLTLSKADYEKHKVYACEVTHQGLSSPVTKSFNRGEC

SEQ ID NO: 175 - protein, 714 aa, synthetic construct
EVQLVESGGGLVQPGGSLRLSCAASGFTFSSYDMSWVRQAPGKRLEWVAFISSGGGSTYYPDTVKGRFTISRDNAKNSLYLQMNSLRAEDTAVYYCGRHYDNYLYAMDYWGQGTLVTVSSASTKGPSVFPLAPSSKSTSGGTAALGCLVKDYFPEPVTVSWNSGALTSGVHTFPAVLQSSGLYSLSSVVTVPSSSLGTQTYICNVNHKPSNTKVDKKVEPKSCGGGGSGGGGSEVQLVESGGGLVQPGGSLRLSCAASGFTFSNYGMSWVRQAPGKCLEWVATISGGGSYTYYPDNLKGRFTISRDNAKNSLYLQMNSLRAEDTAVYYCAAPTAMDYWGQGTLVTVSSGGGGSGGGGSGGGGSGGGGSDIQLTQSPSFLSASVGDRVTITCRASQEISGFLSWLQQKPGKTIKRLIYAASTLDTGVPSRFSGSRSGSEYTLTISSLQPEDFATYYCLQYASYPRTFGCGTKVEIKGGGGSGGGGSESKYGPPCPPCPAPEFLGGPSVFLFPPKPKDTLMISRTPEVTCVVVDVSQEDPEVQFNWYVDGVEVHNAKTKPREEQFNSTYRVVSVLTVLHQDWLNGKEYKCKVSNKGLPSSIEKTISKAKGQPREPQVYTLPPSQEEMTKNQVSLTCLVKGFYPSDIAVEWESNGQPENNYKTTPPVLDSDGSFFLYSRLTVDKSRWQEGNVFSCSVMHEALHNHYTQKSLSLSLGK

SEQ ID NO: 176 - protein, 574 aa, synthetic construct
QVQLVQSGAEVKKPGASVKVSCKGSGYTFTDYTIHWVRQAPGQGLEWMGVISTYQGDASYNQKFKGRATMTVDKSTSTAYMELSSLRSEDTAVYYCARFPDWDYAMDYWGQGTLVTVSSGGGGSGGGGSEVQLVQSGAEVKKPGATVKISCKASGFNIKDTYMHWVQQAPGKGLEWIGRIRPANANAKYDPKFQGRATVTADISTDTAYMELSSLRSEDTAVYYCASYYYGSSGAYWGQGTLVTVSSASTKGPSVFPLAPCSRSTSESTAALGCLVKDYFPEPVTVSWNSGALTSGVHTFPAVLQSSGLYSLSSVVTVPSSSLGTKTYTCNVDHKPSNTKVDKRVESKYGPPCPPCPAPEFLGGPSVFLFPPKPKDTLMISRTPEVTCVVVDVSQEDPEVQFNWYVDGVEVHNAKTKPREEQFNSTYRVVSVLTVLHQDWLNGKEYKCKVSNKGLPSSIEKTISKAKGQPREPQVYTLPPSQEEMTKNQVSLTCLVKGFYPSDIAVEWESNGQPENNYKTTPPVLDSDGSFFLYSRLTVDKSRWQEGNVFSCSVMHEALHNHYTQKSLSLSLGK

SEQ ID NO: 177 - protein, 214 aa, synthetic construct
DIQMTQSPSSLSASVGDRVTITCLASQTIGTWLAWYQQKPGKSPKLLIYAATSLAEGVPSRFSGSGSGTDFTLTISSLQPEDFATYYCQQLYSTPFTFGQGTKVEIKRTVAAPSVFIFPPSDEQLKSGTASVVCLLNNFYPREAKVQWKVDNALQSGNSQESVTEQDSKDSTYSLSSTLTLSKADYEKHKVYACEVTHQGLSSPVTKSFNRGEC

SEQ ID NO: 178 - protein, 214 aa, synthetic construct; identical to SEQ ID NO: 173

SEQ ID NO: 179 - protein, 214 aa, synthetic construct; identical to SEQ ID NO: 119

SEQ ID NO: 180 - protein, 214 aa, synthetic construct; identical to SEQ ID NO: 119

SEQ ID NO: 181 - protein, 214 aa, synthetic construct; identical to SEQ ID NO: 119

SEQ ID NO: 182 - protein, 214 aa, synthetic construct; identical to SEQ ID NO: 119

SEQ ID NO: 183 - protein, 214 aa, synthetic construct; identical to SEQ ID NO: 119

SEQ ID NO: 184 - protein, 214 aa, synthetic construct; identical to SEQ ID NO: 173

SEQ ID NO: 185 - protein, 334 aa, synthetic construct
EIVMTQSPATLSVSPGERATLSCKASQSVDYEGDTYMNWYQQKPGQPPRLLIYAASNLESGIPARFSGSGSGTEFTLTISSLQSEDFAVYYCQQSRELPYTFGQGTKLEIKGGGGSGGGGSEIVMTQSPATLSVSPGERATLSCSVSSSVSYMYWYQQKPGQAPRLLIYDTSSLASGIPARFSGSGSGTEFTLTISSLQSEDFAVYYCQQWSSYPYTFGGGTKVEIKRTVAAPSVFIFPPSDEQLKSGTASVVCLLNNFYPREAKVQWKVDNALQSGNSQESVTEQDSKDSTYSLSSTLTLSKADYEKHKVYACEVTHQGLSSPVTKSFNRGEC

SEQ ID NO: 186 - protein, 334 aa, synthetic construct; identical to SEQ ID NO: 111

SEQ ID NO: 187 - protein, 213 aa, synthetic construct; identical to SEQ ID NO: 124

SEQ ID NO: 188 - protein, 213 aa, synthetic construct; identical to SEQ ID NO: 124

SEQ ID NO: 189 - protein, 213 aa, synthetic construct; identical to SEQ ID NO: 124

SEQ ID NO: 190 - protein, 213 aa, synthetic construct
DIVMTQSPATLSVSPGERATLSCSVSSSVSYMYWYQQKPGQAPRLLIYDTSSLASGIPARFSGSGSGTEFTLTISSLQSEDFAVYYCQQWSSYPYTFGGGTKVEIKRTVAAPSVFIFPPSDEQLKSGTASVVCLLNNFYPREAKVQWKVDNALQSGNSQESVTEQDSKDSTYSLSSTLTLSKADYEKHKVYACEVTHQGLSSPVTKSFNRGEC

SEQ ID NO: 191 - protein, 213 aa, synthetic construct; identical to SEQ ID NO: 190

SEQ ID NO: 192 - protein, 213 aa, synthetic construct; identical to SEQ ID NO: 190

SEQ ID NO: 193 - protein, 714 aa, synthetic construct; identical to SEQ ID NO: 138

SEQ ID NO: 194 - protein, 714 aa, synthetic construct; identical to SEQ ID NO: 138

SEQ ID NO: 195 - protein, 714 aa, synthetic construct
EVQLVESGGGLVQPGGSLRLSCAASGFTFSSYDMSWVRQAPGKRLEWVAFISSGGGSTYYPDTVKGRFTISRDNAKNSLYLQMNSLRAEDTAVYYCGRHYENYLYAMDYWGQGTLVTVSSASTKGPSVFPLAPSSKSTSGGTAALGCLVKDYFPEPVTVSWNSGALTSGVHTFPAVLQSSGLYSLSSVVTVPSSSLGTQTYICNVNHKPSNTKVDKKVEPKSCGGGGSGGGGSEVQLVESGGGLVQPGGSLRLSCAASGFTFSNYGMSWVRQAPGKCLEWVATISGGGSYTYYPDNLKGRFTISRDNAKNSLYLQMNSLRAEDTAVYYCAAPTAMDYWGQGTLVTVSSGGGGSGGGGSGGGGSGGGGSDIQLTQSPSFLSASVGDRVTITCRASQEISGFLSWLQQKPGKTIKRLIYAASTLDSGVPSRFSGSRSGSEYTLTISSLQPEDFATYYCLQYASYPRTFGCGTKVEIKGGGGSGGGGSESKYGPPCPPCPAPEFLGGPSVFLFPPKPKDTLMISRTPEVTCVVVDVSQEDPEVQFNWYVDGVEVHNAKTKPREEQFNSTYRVVSVLTVLHQDWLNGKEYKCKVSNKGLPSSIEKTISKAKGQPREPQVYTLPPSQEEMTKNQVSLTCLVKGFYPSDIAVEWESNGQPENNYKTTPPVLDSDGSFFLYSRLTVDKSRWQEGNVFSCSVMHEALHNHYTQKSLSLSLGK

SEQ ID NO: 196 - protein, 714 aa, synthetic construct
EVQLVESGGGLVQPGGSLRLSCAASGFTFSSYDMSWVRQAPGKRLEWVAFISSGGGSTYYPDTVKGRFTISRDNAKNSLYLQMNSLRAEDTAVYYCGRHYDTYLYAMDYWGQGTLVTVSSASTKGPSVFPLAPSSKSTSGGTAALGCLVKDYFPEPVTVSWNSGALTSGVHTFPAVLQSSGLYSLSSVVTVPSSSLGTQTYICNVNHKPSNTKVDKKVEPKSCGGGGSGGGGSEVQLVESGGGLVQPGGSLRLSCAASGFTFSNYGMSWVRQAPGKCLEWVATISGGGSYTYYPDNLKGRFTISRDNAKNSLYLQMNSLRAEDTAVYYCAAPTAMDYWGQGTLVTVSSGGGGSGGGGSGGGGSGGGGSDIQLTQSPSFLSASVGDRVTITCRASQEISGFLSWLQQKPGKTIKRLIYAASTLDSGVPSRFSGSRSGSEYTLTISSLQPEDFATYYCLQYASYPRTFGCGTKVEIKGGGGSGGGGSESKYGPPCPPCPAPEFLGGPSVFLFPPKPKDTLMISRTPEVTCVVVDVSQEDPEVQFNWYVDGVEVHNAKTKPREEQFNSTYRVVSVLTVLHQDWLNGKEYKCKVSNKGLPSSIEKTISKAKGQPREPQVYTLPPSQEEMTKNQVSLTCLVKGFYPSDIAVEWESNGQPENNYKTTPPVLDSDGSFFLYSRLTVDKSRWQEGNVFSCSVMHEALHNHYTQKSLSLSLGK

SEQ ID NO: 197 - protein, 714 aa, synthetic construct
EVQLVESGGGLVQPGGSLRLSCAASGFTFSSYDMSWVRQAPGKRLEWVAFISSGGGSTYYPDTVKGRFTISRDNAKNSLYLQMNSLRAEDTAVYYCGRHYDAYLYAMDYWGQGTLVTVSSASTKGPSVFPLAPSSKSTSGGTAALGCLVKDYFPEPVTVSWNSGALTSGVHTFPAVLQSSGLYSLSSVVTVPSSSLGTQTYICNVNHKPSNTKVDKKVEPKSCGGGGSGGGGSEVQLVESGGGLVQPGGSLRLSCAASGFTFSNYGMSWVRQAPGKCLEWVATISGGGSYTYYPDNLKGRFTISRDNAKNSLYLQMNSLRAEDTAVYYCAAPTAMDYWGQGTLVTVSSGGGGSGGGGSGGGGSGGGGSDIQLTQSPSFLSASVGDRVTITCRASQEISGFLSWLQQKPGKTIKRLIYAASTLDSGVPSRFSGSRSGSEYTLTISSLQPEDFATYYCLQYASYPRTFGCGTKVEIKGGGGSGGGGSESKYGPPCPPCPAPEFLGGPSVFLFPPKPKDTLMISRTPEVTCVVVDVSQEDPEVQFNWYVDGVEVHNAKTKPREEQFNSTYRVVSVLTVLHQDWLNGKEYKCKVSNKGLPSSIEKTISKAKGQPREPQVYTLPPSQEEMTKNQVSLTCLVKGFYPSDIAVEWESNGQPENNYKTTPPVLDSDGSFFLYSRLTVDKSRWQEGNVFSCSVMHEALHNHYTQKSLSLSLGK

SEQ ID NO: 198 - protein, 714 aa, synthetic construct
EVQLVESGGGLVQPGGSLRLSCAASGFTFSSYDMSWVRQAPGKRLEWVAFISSGGGSTYYPDTVKGRFTISRDNAKNSLYLQMNSLRAEDTAVYYCGRHYDNYLYAMDYWGQGTLVTVSSASTKGPSVFPLAPSSKSTSGGTAALGCLVKDYFPEPVTVSWNSGALTSGVHTFPAVLQSSGLYSLSSVVTVPSSSLGTQTYICNVNHKPSNTKVDKKVEPKSCGGGGSGGGGSEVQLVESGGGLVQPGGSLRLSCAASGFTFSNYGMSWVRQAPGKCLEWVATISGGGSYTYYPDNLKGRFTISRDNAKNSLYLQMNSLRAEDTAVYYCAAPTAMDYWGQGTLVTVSSGGGGSGGGGSGGGGSGGGGSDIQLTQSPSFLSASVGDRVTITCRASQEISGFLSWLQQKPGKTIKRLIYAASTLDAGVPSRFSGSRSGSEYTLTISSLQPEDFATYYCLQYASYPRTFGCGTKVEIKGGGGSGGGGSESKYGPPCPPCPAPEFLGGPSVFLFPPKPKDTLMISRTPEVTCVVVDVSQEDPEVQFNWYVDGVEVHNAKTKPREEQFNSTYRVVSVLTVLHQDWLNGKEYKCKVSNKGLPSSIEKTISKAKGQPREPQVYTLPPSQEEMTKNQVSLTCLVKGFYPSDIAVEWESNGQPENNYKTTPPVLDSDGSFFLYSRLTVDKSRWQEGNVFSCSVMHEALHNHYTQKSLSLSLGK

SEQ ID NO: 199 - protein, 714 aa, synthetic construct; identical to SEQ ID NO: 175

SEQ ID NO: 200 - protein, 714 aa, synthetic construct
EVQLVESGGGLVQPGGSLRLSCAASGFTFSSYDMSWVRQAPGKRLEWVAFISSGGGSTYYPDTVKGRFTISRDNAKNSLYLQMNSLRAEDTAVYYCGRHYDAYLYAMDYWGQGTLVTVSSASTKGPSVFPLAPSSKSTSGGTAALGCLVKDYFPEPVTVSWNSGALTSGVHTFPAVLQSSGLYSLSSVVTVPSSSLGTQTYICNVNHKPSNTKVDKKVEPKSCGGGGSGGGGSEVQLVESGGGLVQPGGSLRLSCAASGFTFSNYGMSWVRQAPGKCLEWVATISGGGSYTYYPDNLKGRFTISRDNAKNSLYLQMNSLRAEDTAVYYCAAPTAMDYWGQGTLVTVSSGGGGSGGGGSGGGGSGGGGSDIQLTQSPSFLSASVGDRVTITCRASQEISGFLSWLQQKPGKTIKRLIYAASTLDTGVPSRFSGSRSGSEYTLTISSLQPEDFATYYCLQYASYPRTFGCGTKVEIKGGGGSGGGGSESKYGPPCPPCPAPEFLGGPSVFLFPPKPKDTLMISRTPEVTCVVVDVSQEDPEVQFNWYVDGVEVHNAKTKPREEQFNSTYRVVSVLTVLHQDWLNGKEYKCKVSNKGLPSSIEKTISKAKGQPREPQVYTLPPSQEEMTKNQVSLTCLVKGFYPSDIAVEWESNGQPENNYKTTPPVLDSDGSFFLYSRLTVDKSRWQEGNVFSCSVMHEALHNHYTQKSLSLSLGK

SEQ ID NO: 201 - protein, 574 aa, synthetic construct; identical to SEQ ID NO: 176

SEQ ID NO: 202 - protein, 574 aa, synthetic construct; identical to SEQ ID NO: 176

SEQ ID NO: 203 - protein, 720 aa, synthetic construct
EVQLVQSGAEVKKPGATVKISCKASGFNIKDTYMHWVQQAPGKGLEWIGRIRPANANAKYDPKFQGRATVTADISTDTAYMELSSLRSEDTAVYYCASYYYGSSGAYWGQGTLVTVSSASTKGPSVFPLAPSSKSTSGGTAALGCLVKDYFPEPVTVSWNSGALTSGVHTFPAVLQSSGLYSLSSVVTVPSSSLGTQTYICNVNHKPSNTKVDKKVEPKSCGGGGSGGGGSEVQLQQSGAELVRPGVSVKISCKGSGYTFTDYTIHWVKQSHAKCLEWIGVISTYQGDASYNQKFKGKATMTVDKSSSTAYMELARLTSEDSAIYYCARFPDWDYAMDYWGQGTSVTVSSGGGGSGGGGSGGGGSGGGGSEIVLTQSPASLAVSLGQRATISCKASQSVDYEGDTYMNWYQQKPGQPPKLLIYAASNLESGVPARFSGSGSGTDFTLNIHPVEEEDAATYYCQHSRELPYTFGCGTKLEIKGGGGSGGGGSESKYGPPCPPCPAPEFLGGPSVFLFPPKPKDTLMISRTPEVTCVVVDVSQEDPEVQFNWYVDGVEVHNAKTKPREEQFNSTYRVVSVLTVLHQDWLNGKEYKCKVSNKGLPSSIEKTISKAKGQPREPQVYTLPPSQEEMTKNQVSLTCLVKGFYPSDIAVEWESNGQPENNYKTTPPVLDSDGSFFLYSRLTVDKSRWQEGNVFSCSVMHEALHNHYTQKSLSLSLGK

SEQ ID NO: 204 - protein, 720 aa, synthetic construct
EVQLVQSGAEVKKPGATVKISCKASGFNIKDTYMHWVQQAPGKGLEWIGRIRPANANAKYDPKFQGRATVTADISTDTAYMELSSLRSEDTAVYYCASYYYGSSGAYWGQGTLVTVSSASTKGPSVFPLAPSSKSTSGGTAALGCLVKDYFPEPVTVSWNSGALTSGVHTFPAVLQSSGLYSLSSVVTVPSSSLGTQTYICNVNHKPSNTKVDKKVEPKSCGGGGSGGGGSEVQLQQSGAELVRPGVSVKISCKGSGYTFTDYTIHWVKQSHAKCLEWIGVISTYQGDASYNQKFKGKATMTVDKSSSTAYMELARLTSEDSAIYYCARFPDWDYAMDYWGQGTSVTVSSGGGGSGGGGSGGGGSGGGGSEIVLTQSPASLAVSLGQRATISCKASQSVDYEGDSYMNWYQQKPGQPPKLLIYAASNLESGVPARFSGSGSGTDFTLNIHPVEEEDAATYYCQHSRELPYTFGCGTKLEIKGGGGSGGGGSESKYGPPCPPCPAPEFLGGPSVFLFPPKPKDTLMISRTPEVTCVVVDVSQEDPEVQFNWYVDGVEVHNAKTKPREEQFNSTYRVVSVLTVLHQDWLNGKEYKCKVSNKGLPSSIEKTISKAKGQPREPQVYTLPPSQEEMTKNQVSLTCLVKGFYPSDIAVEWESNGQPENNYKTTPPVLDSDGSFFLYSRLTVDKSRWQEGNVFSCSVMHEALHNHYTQKSLSLSLGK

SEQ ID NO: 205 - protein, 720 aa, synthetic construct
EVQLVQSGAEVKKPGATVKISCKASGFNIKDTYMHWVQQAPGKGLEWIGRIRPANANAKYDPKFQGRATVTADISTDTAYMELSSLRSEDTAVYYCASYYYGSSGAYWGQGTLVTVSSASTKGPSVFPLAPSSKSTSGGTAALGCLVKDYFPEPVTVSWNSGALTSGVHTFPAVLQSSGLYSLSSVVTVPSSSLGTQTYICNVNHKPSNTKVDKKVEPKSCGGGGSGGGGSEVQLQQSGAELVRPGVSVKISCKGSGYTFTDYTIHWVKQSHAKCLEWIGVISTYQGDASYNQKFKGKATMTVDKSSSTAYMELARLTSEDSAIYYCARFPDWDYAMDYWGQGTSVTVSSGGGGSGGGGSGGGGSGGGGSEIVLTQSPASLAVSLGQRATISCKASQSVDYDGDSYMNWYQQKPGQPPKLLIYAASNLESGVPARFSGSGSGTDFTLNIHPVEEEDAATYYCQHSRELPYTFGCGTKLEIKGGGGSGGGGSESKYGPPCPPCPAPEFLGGPSVFLFPPKPKDTLMISRTPEVTCVVVDVSQEDPEVQFNWYVDGVEVHNAKTKPREEQFNSTYRVVSVLTVLHQDWLNGKEYKCKVSNKGLPSSIEKTISKAKGQPREPQVYTLPPSQEEMTKNQVSLTCLVKGFYPSDIAVEWESNGQPENNYKTTPPVLDSDGSFFLYSRLTVDKSRWQEGNVFSCSVMHEALHNHYTQKSLSLSLGK

SEQ ID NO: 206 - protein, 720 aa, synthetic construct
QVQLVQSGAEVKKPGATVKISCKASGFNIKDTYMHWVQQAPGKGLEWIGRIRPANANAKYDPKFQGRATVTADISTDTAYMELSSLRSEDTAVYYCASYYYGSSGAYWGQGTLVTVSSASTKGPSVFPLAPSSKSTSGGTAALGCLVKDYFPEPVTVSWNSGALTSGVHTFPAVLQSSGLYSLSSVVTVPSSSLGTQTYICNVNHKPSNTKVDKKVEPKSCGGGGSGGGGSEVQLQQSGAELVRPGVSVKISCKGSGYTFTDYTIHWVKQSHAKCLEWIGVISTYQGDASYNQKFKGKATMTVDKSSSTAYMELARLTSEDSAIYYCARFPDWDYAMDYWGQGTSVTVSSGGGGSGGGGSGGGGSGGGGSEIVLTQSPASLAVSLGQRATISCKASQSVDYDGDSYMNWYQQKPGQPPKLLIYAASNLESGVPARFSGSGSGTDFTLNIHPVEEEDAATYYCQHSRELPYTFGCGTKLEIKGGGGSGGGGSESKYGPPCPPCPAPEFLGGPSVFLFPPKPKDTLMISRTPEVTCVVVDVSQEDPEVQFNWYVDGVEVHNAKTKPREEQFNSTYRVVSVLTVLHQDWLNGKEYKCKVSNKGLPSSIEKTISKAKGQPREPQVYTLPPSQEEMTKNQVSLTCLVKGFYPSDIAVEWESNGQPENNYKTTPPVLDSDGSFFLYSRLTVDKSRWQEGNVFSCSVMHEALHNHYTQKSLSLSLGK

SEQ ID NO: 207 - protein, 720 aa, synthetic construct
QVQLVQSGAEVKKPGATVKISCKASGFNIKDTYMHWVQQAPGKGLEWIGRIRPANANAKYDPKFQGRATVTADISTDTAYMELSSLRSEDTAVYYCASYYYGSSGAYWGQGTLVTVSSASTKGPSVFPLAPSSKSTSGGTAALGCLVKDYFPEPVTVSWNSGALTSGVHTFPAVLQSSGLYSLSSVVTVPSSSLGTQTYICNVNHKPSNTKVDKKVEPKSCGGGGSGGGGSEVQLQQSGAELVRPGVSVKISCKGSGYTFTDYTIHWVKQSHAKCLEWIGVISTYQGDASYNQKFKGKATMTVDKSSSTAYMELARLTSEDSAIYYCARFPDWDYALDYWGQGTSVTVSSGGGGSGGGGSGGGGSGGGGSEIVLTQSPASLAVSLGQRATISCKASQSVDYDGDSYMNWYQQKPGQPPKLLIYAASNLESGVPARFSGSGSGTDFTLNIHPVEEEDAATYYCQHSRELPYTFGCGTKLEIKGGGGSGGGGSESKYGPPCPPCPAPEFLGGPSVFLFPPKPKDTLMISRTPEVTCVVVDVSQEDPEVQFNWYVDGVEVHNAKTKPREEQFNSTYRVVSVLTVLHQDWLNGKEYKCKVSNKGLPSSIEKTISKAKGQPREPQVYTLPPSQEEMTKNQVSLTCLVKGFYPSDIAVEWESNGQPENNYKTTPPVLDSDGSFFLYSRLTVDKSRWQEGNVFSCSVMHEALHNHYTQKSLSLSLGK

SEQ ID NO: 208 - protein, 720 aa, synthetic construct
QVQLVQSGAEVKKPGATVKISCKASGFNIKDTYMHWVQQAPGKGLEWIGRIRPANANAKYDPKFQGRATVTADISTDTAYMELSSLRSEDTAVYYCASYYYGSSGAYWGQGTLVTVSSASTKGPSVFPLAPSSKSTSGGTAALGCLVKDYFPEPVTVSWNSGALTSGVHTFPAVLQSSGLYSLSSVVTVPSSSLGTQTYICNVNHKPSNTKVDKKVEPKSCGGGGSGGGGSEVQLQQSGAELVRPGVSVKISCKGSGYTFTDYTIHWVKQSHAKCLEWIGVISTYQGDASYNQKFKGKATMTVDKSSSTAYMELARLTSEDSAIYYCARFPDWDYAVDYWGQGTSVTVSSGGGGSGGGGSGGGGSGGGGSEIVLTQSPASLAVSLGQRATISCKASQSVDYDGDSYMNWYQQKPGQPPKLLIYAASNLESGVPARFSGSGSGTDFTLNIHPVEEEDAATYYCQHSRELPYTFGCGTKLEIKGGGGSGGGGSESKYGPPCPPCPAPEFLGGPSVFLFPPKPKDTLMISRTPEVTCVVVDVSQEDPEVQFNWYVDGVEVHNAKTKPREEQFNSTYRVVSVLTVLHQDWLNGKEYKCKVSNKGLPSSIEKTISKAKGQPREPQVYTLPPSQEEMTKNQVSLTCLVKGFYPSDIAVEWESNGQPENNYKTTPPVLDSDGSFFLYSRLTVDKSRWQEGNVFSCSVMHEALHNHYTQKSLSLSLGK